European Patent Specification EP 3 522 914 B1, published March 8, 2023. Title: Combination treatment for rosacea. Applicant: Micreos Human Health B.V. The sequence listing filed with the application follows.

SEQUENCE LISTING (101 sequences)

SEQ ID NO: 1 - DNA, 1461 bp, Staphylococcus bacteriophage 2638A
atgctaactgctattgactatcttacgaaaaaaggttggaaaatatcatctgaccctcgcacttacgatggttaccctaaaaactacggctacagaaattaccatgaaaacggcattaattatgatgagttttgtggtggttatcatagagcttttgatgtttacagtaacgaaactaacgacgtgcctgctgttactagcggaacagttattgaagcaaacgattacggtaattttggtggtacattcgttattagagacgctaacgataacgattggatatatgggcatctacaacgtggctcaatgcgatttgttgtaggcgacaaagtcaatcaaggtgacattattggtttacaaggtaatagcaactattacgacaatcctatgagtgtacatttacatttacaattacgccctaaagacgcaaagaaagatgaaaaatcacaagtatgtagtggtttggctatggaaaaatatgacattacaaatttaaatgctaaacaagataaatcaaagaatgggagcgtgaaagagttgaaacatatctattcaaaccatattaaaggtaacaagattacagcaccaaaacctagtattcaaggtgtggtcatccacaatgattatggtagtatgacacctagtcaatacttaccatggttatatgcacgtgagaataacggtacacacgttaacggttgggctagtgtttatgcaaatagaaacgaagtgctttggtatcatccgacagactacgtagagtggcattgtggtaatcaatgggcaaatgctaacttaatcggatttgaagtgtgtgagtcgtatcctggtagaatctcggacaaattattcttagaaaatgaagaagcgacattgaaagtagctgcggatgtgatgaagtcgtacggattaccagttaatcgcaacactgtacgtctgcataacgaattcttcggaacttcttgtccacatcgttcgtgggacttgcatgttggcaaaggtgagccttacacaactactaatattaataaaatgaaagactacttcatcaaacgcatcaaacattattatgacggtggaaagctagaagtaagcaaagcagcaactatcaaacaatctgacgttaagcaagaagttaaaaagcaagaagcaaaacaaattgtgaaagcaacagattggaaacagaataaagatggcatttggtataaagctgaacatgcttcgttcacagtgacagcaccagagggaattatcacaagatacaaaggtccttggactggtcacccacaagctggtgtattacaaaaaggtcaaacgattaaatatgatgaggttcaaaaatttgacggtcatgtttgggtatcgtgggaaacgtttgagggcgaaactgtatacatgccggtacgcacatgggacgctaaaactggtaaagttggtaagttgtggggcgaaattaaataa

SEQ ID NO: 2 - protein, 486 aa, Staphylococcus bacteriophage 2638A
MLTAIDYLTKKGWKISSDPRTYDGYPKNYGYRNYHENGINYDEFCGGYHRAFDVYSNETNDVPAVTSGTVIEANDYGNFGGTFVIRDANDNDWIYGHLQRGSMRFVVGDKVNQGDIIGLQGNSNYYDNPMSVHLHLQLRPKDAKKDEKSQVCSGLAMEKYDITNLNAKQDKSKNGSVKELKHIYSNHIKGNKITAPKPSIQGVVIHNDYGSMTPSQYLPWLYARENNGTHVNGWASVYANRNEVLWYHPTDYVEWHCGNQWANANLIGFEVCESYPGRISDKLFLENEEATLKVAADVMKSYGLPVNRNTVRLHNEFFGTSCPHRSWDLHVGKGEPYTTTNINKMKDYFIKRIKHYYDGGKLEVSKAATIKQSDVKQEVKKQEAKQIVKATDWKQNKDGIWYKAEHASFTVTAPEGIITRYKGPWTGHPQAGVLQKGQTIKYDEVQKFDGHVWVSWETFEGETVYMPVRTWDAKTGKVGKLWGEIK

SEQ ID NO: 3 - DNA, 279 bp, Staphylococcus simulans
tggaaaacaaacaaatatggcacactatataaatcagagtcagctagcttcacacctaatacagatataataacaagaacgactggtccatttagaagcatgccgcagtcaggagtcttaaaagcaggtcaaacaattcattatgatgaagtgatgaaacaagacggtcatgtttgggtaggttatacaggtaacagtggccaacgtatttacttgcctgtaagaacatggaataaatctactaatactttaggtgttctttggggaactataaagtga

SEQ ID NO: 4 - protein, 92 aa, Staphylococcus simulans
WKTNKYGTLYKSESASFTPNTDIITRTTGPFRSMPQSGVLKAGQTIHYDEVMKQDGHVWVGYTGNSGQRIYLPVRTWNKSTNTLGVLWGTIK

SEQ ID NO: 5 - DNA, 285 bp, Staphylococcus bacteriophage 2638A
tggaaacagaataaagatggcatttggtataaagctgaacatgcttcgttcacagtgacagcaccagagggaattatcacaagatacaaaggtccttggactggtcacccacaagctggtgtattacaaaaaggtcaaacgattaaatatgatgaggttcaaaaatttgacggtcatgtttgggtatcgtgggaaacgtttgagggcgaaactgtatacatgccggtacgcacatgggacgctaaaactggtaaagttggtaagttgtggggcgaaattaaataa

SEQ ID NO: 6 - protein, 94 aa, Staphylococcus bacteriophage 2638A
WKQNKDGIWYKAEHASFTVTAPEGIITRYKGPWTGHPQAGVLQKGQTIKYDEVQKFDGHVWVSWETFEGETVYMPVRTWDAKTGKVGKLWGEIK

SEQ ID NO: 7 - DNA, 282 bp, Staphylococcus bacteriophage phiNM3
ggtaaatctgcaagtaaaataacagttggaagtaaagcgccttataaccttaaatggtcaaaaggtgcttattttaatgcgaaaatcgacggcttaggtgctacttcagccactagatacggtgataatcgtactaactatagattcgatgttggacaggctgtatacgcgcctggaacattaatatatgtgtttgaaattatagatggttggtgtcgcatttattggaacaatcataatgagtggatatggcatgagagattgattgtgaaagaagtgttt

SEQ ID NO: 8 - protein, 94 aa, Staphylococcus bacteriophage phiNM3
GKSASKITVGSKAPYNLKWSKGAYFNAKIDGLGATSATRYGDNRTNYRFDVGQAVYAPGTLIYVFEIIDGWCRIYWNNHNEWIWHERLIVKEVF

SEQ ID NO: 9 - DNA, 585 bp, Staphylococcus bacteriophage K
atggctaagactcaagcagaaataaataaacgtttagatgcttatgcaaaaggaacagtagatagcccttacagagttaaaaaagctacaagttatgacccatcatttggtgtaatggaagcaggagccattgatgcagatggttactatcacgctcagtgtcaagaccttattacagactatgttttatggttaacagataataaagttagaacttggggtaatgctaaagaccaaattaaacagagttatggtactggatttaaaatacatgaaaataaaccttctactgtacctaaaaaaggttggattgcggtatttacatccggtagttatgaacagtggggtcacataggtattgtatatgatggaggtaatacttctacatttactattttagagcaaaactggaatggttatgctaataaaaaacctacaaaacgtgtagataattattacggattaactcacttcattgaaatacctgtaaaagcaggaactactgttaaaaaagaaacagctaagaaaagcgcaagtaaaacgcctgcacctaaaaagaaagcaacactaaaagtttctaagaat

SEQ ID NO: 10 - protein, 195 aa, Staphylococcus bacteriophage K
MAKTQAEINKRLDAYAKGTVDSPYRVKKATSYDPSFGVMEAGAIDADGYYHAQCQDLITDYVLWLTDNKVRTWGNAKDQIKQSYGTGFKIHENKPSTVPKKGWIAVFTSGSYEQWGHIGIVYDGGNTSTFTILEQNWNGYANKKPTKRVDNYYGLTHFIEIPVKAGTTVKKETAKKSASKTPAPKKKATLKVSKN

SEQ ID NO: 11 - DNA, 420 bp, Staphylococcus bacteriophage Twort
atgaaaaccctgaaacaagcagagtcctacattaagagtaaagtaaatacaggaactgattttgatggtttatatgggtatcagtgtatggacttagcagtagattatatttaccatgtaacagatggtaaaataagaatgtggggtaatgctaaggatgcgataaataactcttttggtggtactgctacggtatataaaaactaccctgcttttagacctaagtacggtgatgtagtcgtatggactactggtaattttgcaacttatggtcatatcgcaatagttactaaccctgacccttatggagaccttcaatatgttacagttcttgaacaaaactggaacggtaacgggatttataaaaccgagttagctacaatcagaacacacgattacacaggaattacacattttatt

SEQ ID NO: 12 - protein, 140 aa, Staphylococcus bacteriophage Twort
MKTLKQAESYIKSKVNTGTDFDGLYGYQCMDLAVDYIYHVTDGKIRMWGNAKDAINNSFGGTATVYKNYPAFRPKYGDVVVWTTGNFATYGHIAIVTNPDPYGDLQYVTVLEQNWNGNGIYKTELATIRTHDYTGITHFI

SEQ ID NO: 13 - DNA, 438 bp, Staphylococcus bacteriophage 2638A
atgctaactgctattgactatcttacgaaaaaaggttggaaaatatcatctgaccctcgcacttacgatggttaccctaaaaactacggctacagaaattaccatgaaaacggcattaattatgatgagttttgtggtggttatcatagagcttttgatgtttacagtaacgaaactaacgacgtgcctgctgttactagcggaacagttattgaagcaaacgattacggtaattttggtggtacattcgttattagagacgctaacgataacgattggatatatgggcatctacaacgtggctcaatgcgatttgttgtaggcgacaaagtcaatcaaggtgacattattggtttacaaggtaatagcaactattacgacaatcctatgagtgtacatttacatttacaattacgccctaaagacgcaaagaaagat

SEQ ID NO: 14 - protein, 146 aa, Staphylococcus bacteriophage 2638A
MLTAIDYLTKKGWKISSDPRTYDGYPKNYGYRNYHENGINYDEFCGGYHRAFDVYSNETNDVPAVTSGTVIEANDYGNFGGTFVIRDANDNDWIYGHLQRGSMRFVVGDKVNQGDIIGLQGNSNYYDNPMSVHLHLQLRPKDAKKD

SEQ ID NO: 15 - DNA, 420 bp, Staphylococcus simulans
gctgcaacacatgaacattcagcacaatggttgaataattacaaaaaaggatatggttacggtccttatccattaggtataaatggcggtatgcactacggagttgatttttttatgaatattggaacaccagtaaaagctatttcaagcggaaaaatagttgaagctggttggagtaattacggaggaggtaatcaaataggtcttattgaaaatgatggagtgcatagacaatggtatatgcatctaagtaaatataatgttaaagtaggagattatgtcaaagctggtcaaataatcggttggtctggaagcactggttattctacagcaccacatttacacttccaaagaatggttaattcattttcaaattcaactgcccaagatccaatgcctttcttaaagagcgcaggatat

SEQ ID NO: 16 - protein, 140 aa, Staphylococcus simulans
AATHEHSAQWLNNYKKGYGYGPYPLGINGGMHYGVDFFMNIGTPVKAISSGKIVEAGWSNYGGGNQIGLIENDGVHRQWYMHLSKYNVKVGDYVKAGQIIGWSGSTGYSTAPHLHFQRMVNSFSNSTAQDPMPFLKSAGY

SEQ ID NO: 17 - DNA, 510 bp, Staphylococcus bacteriophage 2638A
ggtaacaagattacagcaccaaaacctagtattcaaggtgtggtcatccacaatgattatggtagtatgacacctagtcaatacttaccatggttatatgcacgtgagaataacggtacacacgttaacggttgggctagtgtttatgcaaatagaaacgaagtgctttggtatcatccgacagactacgtagagtggcattgtggtaatcaatgggcaaatgctaacttaatcggatttgaagtgtgtgagtcgtatcctggtagaatctcggacaaattattcttagaaaatgaagaagcgacattgaaagtagctgcggatgtgatgaagtcgtacggattaccagttaatcgcaacactgtacgtctgcataacgaattcttcggaacttcttgtccacatcgttcgtgggacttgcatgttggcaaaggtgagccttacacaactactaatattaataaaatgaaagactacttcatcaaacgcatcaaacattattatgacggt

SEQ ID NO: 18 - protein, 169 aa, Staphylococcus bacteriophage 2638A
NKITAPKPSIQGVVIHNDYGSMTPSQYLPWLYARENNGTHVNGWASVYANRNEVLWYHPTDYVEWHCGNQWANANLIGFEVCESYPGRISDKLFLENEEATLKVAADVMKSYGLPVNRNTVRLHNEFFGTSCPHRSWDLHVGKGEPYTTTNINKMKDYFIKRIKHYYDG

SEQ ID NO: 19 - DNA, 1407 bp, artificial
  artificial construct
atggctaagactcaagcagaaataaataaacgtttagatgcttatgcaaaaggaacagtagatagcccttacagagttaaaaaagctacaagttatgacccatcatttggtgtaatggaagcaggagccattgatgcagatggttactatcacgctcagtgtcaagaccttattacagactatgttttatggttaacagataataaagttagaacttggggtaatgctaaagaccaaattaaacagagttatggtactggatttaaaatacatgaaaataaaccttctactgtacctaaaaaaggttggattgcggtatttacatccggtagttatgaacagtggggtcacataggtattgtatatgatggaggtaatacttctacatttactattttagagcaaaactggaatggttatgctaataaaaaacctacaaaacgtgtagataattattacggattaactcacttcattgaaatacctgtaaaagcaggaactactgttaaaaaagaaacagctaagaaaagcgcaagtaaaacgcctgcacctaaaaagaaagcaacactaaaagtttctaagaatgagctcatggctaagactcaagcagaaataaataaacgtttagatgcttatgcaaaaggaacagtagatagcccttacagagttaaaaaagctacaagttatgacccatcatttggtgtaatggaagcaggagccattgatgcagatggttactatcacgctcagtgtcaagaccttattacagactatgttttatggttaacagataataaagttagaacttggggtaatgctaaagaccaaattaaacagagttatggtactggatttaaaatacatgaaaataaaccttctactgtacctaaaaaaggttggattgcggtatttacatccggtagttatgaacagtggggtcacataggtattgtatatgatggaggtaatacttctacatttactattttagagcaaaactggaatggttatgctaataaaaaacctacaaaacgtgtagataattattacggattaactcacttcattgaaatacctgtaaaagcaggaaaagcaggtggtacagtaactccaacgccgaatacaggttggaaaacaaacaaatatggcacactatataaatcagagtcagctagcttcacacctaatacagatataataacaagaacgactggtccatttagaagcatgccgcagtcaggagtcttaaaagcaggtcaaacaattcattatgatgaagtgatgaaacaagacggtcatgtttgggtaggttatacaggtaacagtggccaacgtatttacttgcctgtaagaacatggaataaatctactaatactttaggtgttctttggggaactataaagtaa

SEQ ID NO: 20 - protein, 468 aa, artificial
  artificial construct
MAKTQAEINKRLDAYAKGTVDSPYRVKKATSYDPSFGVMEAGAIDADGYYHAQCQDLITDYVLWLTDNKVRTWGNAKDQIKQSYGTGFKIHENKPSTVPKKGWIAVFTSGSYEQWGHIGIVYDGGNTSTFTILEQNWNGYANKKPTKRVDNYYGLTHFIEIPVKAGTTVKKETAKKSASKTPAPKKKATLKVSKNELMAKTQAEINKRLDAYAKGTVDSPYRVKKATSYDPSFGVMEAGAIDADGYYHAQCQDLITDYVLWLTDNKVRTWGNAKDQIKQSYGTGFKIHENKPSTVPKKGWIAVFTSGSYEQWGHIGIVYDGGNTSTFTILEQNWNGYANKKPTKRVDNYYGLTHFIEIPVKAGKAGGTVTPTPNTGWKTNKYGTLYKSESASFTPNTDIITRTTGPFRSMPQSGVLKAGQTIHYDEVMKQDGHVWVGYTGNSGQRIYLPVRTWNKSTNTLGVLWGTIK

SEQ ID NO: 21 - DNA, 1209 bp, artificial
  artificial construct
gctgcaacacatgaacattcagcacaatggttgaataattacaaaaaaggatatggttacggtccttatccattaggtataaatggcggtatgcactacggagttgatttttttatgaatattggaacaccagtaaaagctatttcaagcggaaaaatagttgaagctggttggagtaattacggaggaggtaatcaaataggtcttattgaaaatgatggagtgcatagacaatggtatatgcatctaagtaaatataatgttaaagtaggagattatgtcaaagctggtcaaataatcggttggtctggaagcactggttattctacagcaccacatttacacttccaaagaatggttaattcattttcaaattcaactgcccaagatccaatgcctttcttaaagagcgcaggatatggaaaagcaggtggtacagtaactccaacgccgaatacaggtgagctcgctgcaacacatgaacattcagcacaatggttgaataattacaaaaaaggatatggttacggtccttatccattaggtataaatggcggtatgcactacggagttgatttttttatgaatattggaacaccagtaaaagctatttcaagcggaaaaatagttgaagctggttggagtaattacggaggaggtaatcaaataggtcttattgaaaatgatggagtgcatagacaatggtatatgcatctaagtaaatataatgttaaagtaggagattatgtcaaagctggtcaaataatcggttggtctggaagcactggttattctacagcaccacatttacacttccaaagaatggttaattcattttcaaattcaactgcccaagatccaatgcctttcttaaagagcgcaggatatggaaaagcaggtggtacagtaactccaacgccgaatacaggttggaaaacaaacaaatatggcacactatataaatcagagtcagctagcttcacacctaatacagatataataacaagaacgactggtccatttagaagcatgccgcagtcaggagtcttaaaagcaggtcaaacaattcattatgatgaagtgatgaaacaagacggtcatgtttgggtaggttatacaggtaacagtggccaacgtatttacttgcctgtaagaacatggaataaatctactaatactttaggtgttctttggggaactataaagtaa

SEQ ID NO: 22 - protein, 402 aa, artificial
  artificial construct
AATHEHSAQWLNNYKKGYGYGPYPLGINGGMHYGVDFFMNIGTPVKAISSGKIVEAGWSNYGGGNQIGLIENDGVHRQWYMHLSKYNVKVGDYVKAGQIIGWSGSTGYSTAPHLHFQRMVNSFSNSTAQDPMPFLKSAGYGKAGGTVTPTPNTGELAATHEHSAQWLNNYKKGYGYGPYPLGINGGMHYGVDFFMNIGTPVKAISSGKIVEAGWSNYGGGNQIGLIENDGVHRQWYMHLSKYNVKVGDYVKAGQIIGWSGSTGYSTAPHLHFQRMVNSFSNSTAQDPMPFLKSAGYGKAGGTVTPTPNTGWKTNKYGTLYKSESASFTPNTDIITRTTGPFRSMPQSGVLKAGQTIHYDEVMKQDGHVWVGYTGNSGQRIYLPVRTWNKSTNTLGVLWGTIK

SEQ ID NO: 23 - DNA, 1686 bp, artificial
  artificial construct
gcaaagaaagatgaaaaatcacaagtatgtagtggtttggctatggaaaaatatgacattacaaatttaaatgctaaacaagataaatcaaagaatgggagcgtgaaagagttgaaacatatctattcaaaccatattaaaggtaacaagattacagcaccaaaacctagtattcaaggtgtggtcatccacaatgattatggtagtatgacacctagtcaatacttaccatggttatatgcacgtgagaataacggtacacacgttaacggttgggctagtgtttatgcaaatagaaacgaagtgctttggtatcatccgacagactacgtagagtggcattgtggtaatcaatgggcaaatgctaacttaatcggatttgaagtgtgtgagtcgtatcctggtagaatctcggacaaattattcttagaaaatgaagaagcgacattgaaagtagctgcggatgtgatgaagtcgtacggattaccagttaatcgcaacactgtacgtctgcataacgaattcttcggaacttcttgtccacatcgttcgtgggacttgcatgttggcaaaggtgagccttacacaactactaatattaataaaatgaaagactacttcatcaaacgcatcaaacattattatgacggtgagctcgcaaagaaagatgaaaaatcacaagtatgtagtggtttggctatggaaaaatatgacattacaaatttaaatgctaaacaagataaatcaaagaatgggagcgtgaaagagttgaaacatatctattcaaaccatattaaaggtaacaagattacagcaccaaaacctagtattcaaggtgtggtcatccacaatgattatggtagtatgacacctagtcaatacttaccatggttatatgcacgtgagaataacggtacacacgttaacggttgggctagtgtttatgcaaatagaaacgaagtgctttggtatcatccgacagactacgtagagtggcattgtggtaatcaatgggcaaatgctaacttaatcggatttgaagtgtgtgagtcgtatcctggtagaatctcggacaaattattcttagaaaatgaagaagcgacattgaaagtagctgcggatgtgatgaagtcgtacggattaccagttaatcgcaacactgtacgtctgcataacgaattcttcggaacttcttgtccacatcgttcgtgggacttgcatgttggcaaaggtgagccttacacaactactaatattaataaaatgaaagactacttcatcaaacgcatcaaacattattatgacggtggaaagctagaagtaagcaaagcagcaactatcaaacaatctgacgttaagcaagaagttaaaaagcaagaagcaaaacaaattgtgaaagcaacagattggaaaacaaacaaatatggcacactatataaatcagagtcagctagcttcacacctaatacagatataataacaagaacgactggtccatttagaagcatgccgcagtcaggagtcttaaaagcaggtcaaacaattcattatgatgaagtgatgaaacaagacggtcatgtttgggtaggttatacaggtaacagtggccaacgtatttacttgcctgtaagaacatggaataaatctactaatactttaggtgttctttggggaactataaagtaa

SEQ ID NO: 24 - protein, 561 aa, artificial
  artificial construct
AKKDEKSQVCSGLAMEKYDITNLNAKQDKSKNGSVKELKHIYSNHIKGNKITAPKPSIQGVVIHNDYGSMTPSQYLPWLYARENNGTHVNGWASVYANRNEVLWYHPTDYVEWHCGNQWANANLIGFEVCESYPGRISDKLFLENEEATLKVAADVMKSYGLPVNRNTVRLHNEFFGTSCPHRSWDLHVGKGEPYTTTNINKMKDYFIKRIKHYYDGELAKKDEKSQVCSGLAMEKYDITNLNAKQDKSKNGSVKELKHIYSNHIKGNKITAPKPSIQGVVIHNDYGSMTPSQYLPWLYARENNGTHVNGWASVYANRNEVLWYHPTDYVEWHCGNQWANANLIGFEVCESYPGRISDKLFLENEEATLKVAADVMKSYGLPVNRNTVRLHNEFFGTSCPHRSWDLHVGKGEPYTTTNINKMKDYFIKRIKHYYDGGKLEVSKAATIKQSDVKQEVKKQEAKQIVKATDWKTNKYGTLYKSESASFTPNTDIITRTTGPFRSMPQSGVLKAGQTIHYDEVMKQDGHVWVGYTGNSGQRIYLPVRTWNKSTNTLGVLWGTIK

SEQ ID NO: 25 - DNA, 1131 bp, artificial
  artificial construct
atgagaggatcgcatcaccatcaccatcacggatctggctctggatctggtatcgagggaaggccttataatggaactggatccgcatgcgagctcgcaaagaaagatgaaaaatcacaagtatgtagtggtttggctatggaaaaatatgacattacaaatttaaatgctaaacaagataaatcaaagaatgggagcgtgaaagagttgaaacatatctattcaaaccatattaaaggtaacaagattacagcaccaaaacctagtattcaaggtgtggtcatccacaatgattatggtagtatgacacctagtcaatacttaccatggttatatgcacgtgagaataacggtacacacgttaacggttgggctagtgtttatgcaaatagaaacgaagtgctttggtatcatccgacagactacgtagagtggcattgtggtaatcaatgggcaaatgctaacttaatcggatttgaagtgtgtgagtcgtatcctggtagaatctcggacaaattattcttagaaaatgaagaagcgacattgaaagtagctgcggatgtgatgaagtcgtacggattaccagttaatcgcaacactgtacgtctgcataacgaattcttcggaacttcttgtccacatcgttcgtgggacttgcatgttggcaaaggtgagccttacacaactactaatattaataaaatgaaagactacttcatcaaacgcatcaaacattattatgacggtggaaagctagaagtaagcaaagcagcaactatcaaacaatctgacgttaagcaagaagttaaaaagcaagaagcaaaacaaattgtgaaagcaacagattggaaacagaataaagatggcatttggtataaagctgaacatgcttcgttcacagtgacagcaccagagggaattatcacaagatacaaaggtccttggactggtcacccacaagctggtgtattacaaaaaggtcaaacgattaaatatgatgaggttcaaaaatttgacggtcatgtttgggtatcgtgggaaacgtttgagggcgaaactgtatacatgccggtacgcacatgggacgctaaaactggtaaagttggtaagttgtggggcgaaattaaataa

SEQ ID NO: 26 - protein, 376 aa, artificial
  artificial construct
MRGSHHHHHHGSGSGSGIEGRPYNGTGSACELAKKDEKSQVCSGLAMEKYDITNLNAKQDKSKNGSVKELKHIYSNHIKGNKITAPKPSIQGVVIHNDYGSMTPSQYLPWLYARENNGTHVNGWASVYANRNEVLWYHPTDYVEWHCGNQWANANLIGFEVCESYPGRISDKLFLENEEATLKVAADVMKSYGLPVNRNTVRLHNEFFGTSCPHRSWDLHVGKGEPYTTTNINKMKDYFIKRIKHYYDGGKLEVSKAATIKQSDVKQEVKKQEAKQIVKATDWKQNKDGIWYKAEHASFTVTAPEGIITRYKGPWTGHPQAGVLQKGQTIKYDEVQKFDGHVWVSWETFEGETVYMPVRTWDAKTGKVGKLWGEIK

SEQ ID NO: 27 - DNA, 1125 bp, artificial
  artificial construct
atgagaggatcgcatcaccatcaccatcacggatctggctctggatctggtatcgagggaaggccttataatggaactggatccgcatgcgagctcgcaaagaaagatgaaaaatcacaagtatgtagtggtttggctatggaaaaatatgacattacaaatttaaatgctaaacaagataaatcaaagaatgggagcgtgaaagagttgaaacatatctattcaaaccatattaaaggtaacaagattacagcaccaaaacctagtattcaaggtgtggtcatccacaatgattatggtagtatgacacctagtcaatacttaccatggttatatgcacgtgagaataacggtacacacgttaacggttgggctagtgtttatgcaaatagaaacgaagtgctttggtatcatccgacagactacgtagagtggcattgtggtaatcaatgggcaaatgctaacttaatcggatttgaagtgtgtgagtcgtatcctggtagaatctcggacaaattattcttagaaaatgaagaagcgacattgaaagtagctgcggatgtgatgaagtcgtacggattaccagttaatcgcaacactgtacgtctgcataacgaattcttcggaacttcttgtccacatcgttcgtgggacttgcatgttggcaaaggtgagccttacacaactactaatattaataaaatgaaagactacttcatcaaacgcatcaaacattattatgacggtggaaagctagaagtaagcaaagcagcaactatcaaacaatctgacgttaagcaagaagttaaaaagcaagaagcaaaacaaattgtgaaagcaacagattggaaaacaaacaaatatggcacactatataaatcagagtcagctagcttcacacctaatacagatataataacaagaacgactggtccatttagaagcatgccgcagtcaggagtcttaaaagcaggtcaaacaattcattatgatgaagtgatgaaacaagacggtcatgtttgggtaggttatacaggtaacagtggccaacgtatttacttgcctgtaagaacatggaataaatctactaatactttaggtgttctttggggaactataaagtaa

SEQ ID NO: 28 - protein, 374 aa, artificial
  artificial construct
MRGSHHHHHHGSGSGSGIEGRPYNGTGSACELAKKDEKSQVCSGLAMEKYDITNLNAKQDKSKNGSVKELKHIYSNHIKGNKITAPKPSIQGVVIHNDYGSMTPSQYLPWLYARENNGTHVNGWASVYANRNEVLWYHPTDYVEWHCGNQWANANLIGFEVCESYPGRISDKLFLENEEATLKVAADVMKSYGLPVNRNTVRLHNEFFGTSCPHRSWDLHVGKGEPYTTTNINKMKDYFIKRIKHYYDGGKLEVSKAATIKQSDVKQEVKKQEAKQIVKATDWKTNKYGTLYKSESASFTPNTDIITRTTGPFRSMPQSGVLKAGQTIHYDEVMKQDGHVWVGYTGNSGQRIYLPVRTWNKSTNTLGVLWGTIK

SEQ ID NO: 29 - DNA, 1131 bp, artificial
  artificial construct
atgagaggatcgcatcaccatcaccatcacggatctggctctggatctggtatcgagggaaggccttataatggaactggatccgcatgcgagctcgcaaagaaagatgaaaaatcacaagtatgtagtggtttggctatggaaaaatatgacattacaaatttaaatgctaaacaagataaatcaaagaatgggagcgtgaaagagttgaaacatatctattcaaaccatattaaaggtaacaagattacagcaccaaaacctagtattcaaggtgtggtcatccacaatgattatggtagtatgacacctagtcaatacttaccatggttatatgcacgtgagaataacggtacacacgttaacggttgggctagtgtttatgcaaatagaaacgaagtgctttggtatcatccgacagactacgtagagtggcattgtggtaatcaatgggcaaatgctaacttaatcggatttgaagtgtgtgagtcgtatcctggtagaatctcggacaaattattcttagaaaatgaagaagcgacattgaaagtagctgcggatgtgatgaagtcgtacggattaccagttaatcgcaacactgtacgtctgcataacgaattcttcggaacttcttgtccacatcgttcgtgggacttgcatgttggcaaaggtgagccttacacaactactaatattaataaaatgaaagactacttcatcaaacgcatcaaacattattatgacggtggaaagctagaagtaagcaaagcagcaactatcaaacaatctgacgttaagcaagaagttaaaaagcaagaagcaaaacaaattgtgaaagcaacagatggtaaatctgcaagtaaaataacagttggaagtaaagcgccttataaccttaaatggtcaaaaggtgcttattttaatgcgaaaatcgacggcttaggtgctacttcagccactagatacggtgataatcgtactaactatagattcgatgttggacaggctgtatacgcgcctggaacattaatatatgtgtttgaaattatagatggttggtgtcgcatttattggaacaatcataatgagtggatatggcatgagagattgattgtgaaagaagtgttttaa

SEQ ID NO: 30 - protein, 376 aa, artificial
  artificial construct
MRGSHHHHHHGSGSGSGIEGRPYNGTGSACELAKKDEKSQVCSGLAMEKYDITNLNAKQDKSKNGSVKELKHIYSNHIKGNKITAPKPSIQGVVIHNDYGSMTPSQYLPWLYARENNGTHVNGWASVYANRNEVLWYHPTDYVEWHCGNQWANANLIGFEVCESYPGRISDKLFLENEEATLKVAADVMKSYGLPVNRNTVRLHNEFFGTSCPHRSWDLHVGKGEPYTTTNINKMKDYFIKRIKHYYDGGKLEVSKAATIKQSDVKQEVKKQEAKQIVKATDGKSASKITVGSKAPYNLKWSKGAYFNAKIDGLGATSATRYGDNRTNYRFDVGQAVYAPGTLIYVFEIIDGWCRIYWNNHNEWIWHERLIVKEVF

SEQ ID NO: 31 - DNA, 975 bp, artificial
  artificial construct
atgagaggatcgcatcaccatcaccatcacggatctggctctggatctggtatcgagggaaggccttataatggaactggatccgcatgcgagctcatggctaagactcaagcagaaataaataaacgtttagatgcttatgcaaaaggaacagtagatagcccttacagagttaaaaaagctacaagttatgacccatcatttggtgtaatggaagcaggagccattgatgcagatggttactatcacgctcagtgtcaagaccttattacagactatgttttatggttaacagataataaagttagaacttggggtaatgctaaagaccaaattaaacagagttatggtactggatttaaaatacatgaaaataaaccttctactgtacctaaaaaaggttggattgcggtatttacatccggtagttatgaacagtggggtcacataggtattgtatatgatggaggtaatacttctacatttactattttagagcaaaactggaatggttatgctaataaaaaacctacaaaacgtgtagataattattacggattaactcacttcattgaaatacctgtaaaagcaggaaagctagaagtaagcaaagcagcaactatcaaacaatctgacgttaagcaagaagttaaaaagcaagaagcaaaacaaattgtgaaagcaacagattggaaacagaataaagatggcatttggtataaagctgaacatgcttcgttcacagtgacagcaccagagggaattatcacaagatacaaaggtccttggactggtcacccacaagctggtgtattacaaaaaggtcaaacgattaaatatgatgaggttcaaaaatttgacggtcatgtttgggtatcgtgggaaacgtttgagggcgaaactgtatacatgccggtacgcacatgggacgctaaaactggtaaagttggtaagttgtggggcgaaattaaataa

SEQ ID NO: 32 - protein, 324 aa, artificial
  artificial construct
MRGSHHHHHHGSGSGSGIEGRPYNGTGSACELMAKTQAEINKRLDAYAKGTVDSPYRVKKATSYDPSFGVMEAGAIDADGYYHAQCQDLITDYVLWLTDNKVRTWGNAKDQIKQSYGTGFKIHENKPSTVPKKGWIAVFTSGSYEQWGHIGIVYDGGNTSTFTILEQNWNGYANKKPTKRVDNYYGLTHFIEIPVKAGKLEVSKAATIKQSDVKQEVKKQEAKQIVKATDWKQNKDGIWYKAEHASFTVTAPEGIITRYKGPWTGHPQAGVLQKGQTIKYDEVQKFDGHVWVSWETFEGETVYMPVRTWDAKTGKVGKLWGEIK

SEQ ID NO: 33 - DNA, 912 bp, artificial
  artificial construct
atgagaggatcgcatcaccatcaccatcacggatctggctctggatctggtatcgagggaaggccttataatggaactggatccgcatgcgagctcatggctaagactcaagcagaaataaataaacgtttagatgcttatgcaaaaggaacagtagatagcccttacagagttaaaaaagctacaagttatgacccatcatttggtgtaatggaagcaggagccattgatgcagatggttactatcacgctcagtgtcaagaccttattacagactatgttttatggttaacagataataaagttagaacttggggtaatgctaaagaccaaattaaacagagttatggtactggatttaaaatacatgaaaataaaccttctactgtacctaaaaaaggttggattgcggtatttacatccggtagttatgaacagtggggtcacataggtattgtatatgatggaggtaatacttctacatttactattttagagcaaaactggaatggttatgctaataaaaaacctacaaaacgtgtagataattattacggattaactcacttcattgaaatacctgtaaaagcaggaaaagcaggtggtacagtaactccaacgccgaatacaggttggaaaacaaacaaatatggcacactatataaatcagagtcagctagcttcacacctaatacagatataataacaagaacgactggtccatttagaagcatgccgcagtcaggagtcttaaaagcaggtcaaacaattcattatgatgaagtgatgaaacaagacggtcatgtttgggtaggttatacaggtaacagtggccaacgtatttacttgcctgtaagaacatggaataaatctactaatactttaggtgttctttggggaactataaagtaa

SEQ ID NO: 34 - protein, 303 aa, artificial
  artificial construct
MRGSHHHHHHGSGSGSGIEGRPYNGTGSACELMAKTQAEINKRLDAYAKGTVDSPYRVKKATSYDPSFGVMEAGAIDADGYYHAQCQDLITDYVLWLTDNKVRTWGNAKDQIKQSYGTGFKIHENKPSTVPKKGWIAVFTSGSYEQWGHIGIVYDGGNTSTFTILEQNWNGYANKKPTKRVDNYYGLTHFIEIPVKAGKAGGTVTPTPNTGWKTNKYGTLYKSESASFTPNTDIITRTTGPFRSMPQSGVLKAGQTIHYDEVMKQDGHVWVGYTGNSGQRIYLPVRTWNKSTNTLGVLWGTIK

SEQ ID NO: 35 - DNA, 966 bp, artificial
  artificial construct
atgagaggatcgcatcaccatcaccatcacggatctggctctggatctggtatcgagggaaggccttataatggaactggatccgcatgcgagctcatggctaagactcaagcagaaataaataaacgtttagatgcttatgcaaaaggaacagtagatagcccttacagagttaaaaaagctacaagttatgacccatcatttggtgtaatggaagcaggagccattgatgcagatggttactatcacgctcagtgtcaagaccttattacagactatgttttatggttaacagataataaagttagaacttggggtaatgctaaagaccaaattaaacagagttatggtactggatttaaaatacatgaaaataaaccttctactgtacctaaaaaaggttggattgcggtatttacatccggtagttatgaacagtggggtcacataggtattgtatatgatggaggtaatacttctacatttactattttagagcaaaactggaatggttatgctaataaaaaacctacaaaacgtgtagataattattacggattaactcacttcattgaaatacctgtaaaagcaggaactactgttaaaaaagaaacagctaagaaaagcgcaagtaaaacgcctgcacctaaaaagaaagcaacactaaaagtttctaagaatggtaaatctgcaagtaaaataacagttggaagtaaagcgccttataaccttaaatggtcaaaaggtgcttattttaatgcgaaaatcgacggcttaggtgctacttcagccactagatacggtgataatcgtactaactatagattcgatgttggacaggctgtatacgcgcctggaacattaatatatgtgtttgaaattatagatggttggtgtcgcatttattggaacaatcataatgagtggatatggcatgagagattgattgtgaaagaagtgttttaa

SEQ ID NO: 36 - protein, 321 aa, artificial
  artificial construct
MRGSHHHHHHGSGSGSGIEGRPYNGTGSACELMAKTQAEINKRLDAYAKGTVDSPYRVKKATSYDPSFGVMEAGAIDADGYYHAQCQDLITDYVLWLTDNKVRTWGNAKDQIKQSYGTGFKIHENKPSTVPKKGWIAVFTSGSYEQWGHIGIVYDGGNTSTFTILEQNWNGYANKKPTKRVDNYYGLTHFIEIPVKAGTTVKKETAKKSASKTPAPKKKATLKVSKNGKSASKITVGSKAPYNLKWSKGAYFNAKIDGLGATSATRYGDNRTNYRFDVGQAVYAPGTLIYVFEIIDGWCRIYWNNHNEWIWHERLIVKEVF

SEQ ID NO: 37 - DNA, 927 bp, artificial
  artificial construct
atgagaggatcgcatcaccatcaccatcacggatctggctctggatctggtatcgagggaaggccttataatggaactggatccgcatgcgagctcatgaaaaccctgaaacaagcagagtcctacattaagagtaaagtaaatacaggaactgattttgatggtttatatgggtatcagtgtatggacttagcagtagattatatttaccatgtaacagatggtaaaataagaatgtggggtaatgctaaggatgcgataaataactcttttggtggtactgctacggtatataaaaactaccctgcttttagacctaagtacggtgatgtagtcgtatggactactggtaattttgcaacttatggtcatatcgcaatagttactaaccctgacccttatggagaccttcaatatgttacagttcttgaacaaaactggaacggtaacgggatttataaaaccgagttagctacaatcagaacacacgattacacaggaattacacattttattagacctaactttgctactgaatcaagtgtaaaaaagaaagatacaaagaaaaaaccaaaaccatcaaatagagatggaataaataaagataaaattgtatatgatagaactaatattaattacaattggaaacagaataaagatggcatttggtataaagctgaacatgcttcgttcacagtgacagcaccagagggaattatcacaagatacaaaggtccttggactggtcacccacaagctggtgtattacaaaaaggtcaaacgattaaatatgatgaggttcaaaaatttgacggtcatgtttgggtatcgtgggaaacgtttgagggcgaaactgtatacatgccggtacgcacatgggacgctaaaactggtaaagttggtaagttgtggggcgaaattaaataa

SEQ ID NO: 38 - protein, 308 aa, artificial
  artificial construct
MRGSHHHHHHGSGSGSGIEGRPYNGTGSACELMKTLKQAESYIKSKVNTGTDFDGLYGYQCMDLAVDYIYHVTDGKIRMWGNAKDAINNSFGGTATVYKNYPAFRPKYGDVVVWTTGNFATYGHIAIVTNPDPYGDLQYVTVLEQNWNGNGIYKTELATIRTHDYTGITHFIRPNFATESSVKKKDTKKKPKPSNRDGINKDKIVYDRTNINYNWKQNKDGIWYKAEHASFTVTAPEGIITRYKGPWTGHPQAGVLQKGQTIKYDEVQKFDGHVWVSWETFEGETVYMPVRTWDAKTGKVGKLWGEIK

SEQ ID NO: 39 - DNA, 921 bp, artificial
  artificial construct
atgagaggatcgcatcaccatcaccatcacggatctggctctggatctggtatcgagggaaggccttataatggaactggatccgcatgcgagctcatgaaaaccctgaaacaagcagagtcctacattaagagtaaagtaaatacaggaactgattttgatggtttatatgggtatcagtgtatggacttagcagtagattatatttaccatgtaacagatggtaaaataagaatgtggggtaatgctaaggatgcgataaataactcttttggtggtactgctacggtatataaaaactaccctgcttttagacctaagtacggtgatgtagtcgtatggactactggtaattttgcaacttatggtcatatcgcaatagttactaaccctgacccttatggagaccttcaatatgttacagttcttgaacaaaactggaacggtaacgggatttataaaaccgagttagctacaatcagaacacacgattacacaggaattacacattttattagacctaactttgctactgaatcaagtgtaaaaaagaaagatacaaagaaaaaaccaaaaccatcaaatagagatggaataaataaagataaaattgtatatgatagaactaatattaattacaattggaaaacaaacaaatatggcacactatataaatcagagtcagctagcttcacacctaatacagatataataacaagaacgactggtccatttagaagcatgccgcagtcaggagtcttaaaagcaggtcaaacaattcattatgatgaagtgatgaaacaagacggtcatgtttgggtaggttatacaggtaacagtggccaacgtatttacttgcctgtaagaacatggaataaatctactaatactttaggtgttctttggggaactataaagtaa

SEQ ID NO: 40 - protein, 306 aa, artificial
  artificial construct
MRGSHHHHHHGSGSGSGIEGRPYNGTGSACELMKTLKQAESYIKSKVNTGTDFDGLYGYQCMDLAVDYIYHVTDGKIRMWGNAKDAINNSFGGTATVYKNYPAFRPKYGDVVVWTTGNFATYGHIAIVTNPDPYGDLQYVTVLEQNWNGNGIYKTELATIRTHDYTGITHFIRPNFATESSVKKKDTKKKPKPSNRDGINKDKIVYDRTNINYNWKTNKYGTLYKSESASFTPNTDIITRTTGPFRSMPQSGVLKAGQTIHYDEVMKQDGHVWVGYTGNSGQRIYLPVRTWNKSTNTLGVLWGTIK

SEQ ID NO: 41 - DNA, 927 bp, artificial
  artificial construct
atgagaggatcgcatcaccatcaccatcacggatctggctctggatctggtatcgagggaaggccttataatggaactggatccgcatgcgagctcatgaaaaccctgaaacaagcagagtcctacattaagagtaaagtaaatacaggaactgattttgatggtttatatgggtatcagtgtatggacttagcagtagattatatttaccatgtaacagatggtaaaataagaatgtggggtaatgctaaggatgcgataaataactcttttggtggtactgctacggtatataaaaactaccctgcttttagacctaagtacggtgatgtagtcgtatggactactggtaattttgcaacttatggtcatatcgcaatagttactaaccctgacccttatggagaccttcaatatgttacagttcttgaacaaaactggaacggtaacgggatttataaaaccgagttagctacaatcagaacacacgattacacaggaattacacattttattagacctaactttgctactgaatcaagtgtaaaaaagaaagatacaaagaaaaaaccaaaaccatcaaatagagatggaataaataaagataaaattgtatatgatagaactaatattaattacaatggtaaatctgcaagtaaaataacagttggaagtaaagcgccttataaccttaaatggtcaaaaggtgcttattttaatgcgaaaatcgacggcttaggtgctacttcagccactagatacggtgataatcgtactaactatagattcgatgttggacaggctgtatacgcgcctggaacattaatatatgtgtttgaaattatagatggttggtgtcgcatttattggaacaatcataatgagtggatatggcatgagagattgattgtgaaagaagtgttttaa

SEQ ID NO: 42 - protein, 308 aa, artificial
  artificial construct
MRGSHHHHHHGSGSGSGIEGRPYNGTGSACELMKTLKQAESYIKSKVNTGTDFDGLYGYQCMDLAVDYIYHVTDGKIRMWGNAKDAINNSFGGTATVYKNYPAFRPKYGDVVVWTTGNFATYGHIAIVTNPDPYGDLQYVTVLEQNWNGNGIYKTELATIRTHDYTGITHFIRPNFATESSVKKKDTKKKPKPSNRDGINKDKIVYDRTNINYNGKSASKITVGSKAPYNLKWSKGAYFNAKIDGLGATSATRYGDNRTNYRFDVGQAVYAPGTLIYVFEIIDGWCRIYWNNHNEWIWHERLIVKEVF

SEQ ID NO: 43 - DNA, 843 bp, artificial
  artificial construct
atgagaggatcgcatcaccatcaccatcacggatctggctctggatctggtatcgagggaaggccttataatggaactggatccgcatgcgagctcgctgcaacacatgaacattcagcacaatggttgaataattacaaaaaaggatatggttacggtccttatccattaggtataaatggcggtatgcactacggagttgatttttttatgaatattggaacaccagtaaaagctatttcaagcggaaaaatagttgaagctggttggagtaattacggaggaggtaatcaaataggtcttattgaaaatgatggagtgcatagacaatggtatatgcatctaagtaaatataatgttaaagtaggagattatgtcaaagctggtcaaataatcggttggtctggaagcactggttattctacagcaccacatttacacttccaaagaatggttaattcattttcaaattcaactgcccaagatccaatgcctttcttaaagagcgcaggatatggaaaagcaggtggtacagtaactccaacgccgaatacaggttggaaacagaataaagatggcatttggtataaagctgaacatgcttcgttcacagtgacagcaccagagggaattatcacaagatacaaaggtccttggactggtcacccacaagctggtgtattacaaaaaggtcaaacgattaaatatgatgaggttcaaaaatttgacggtcatgtttgggtatcgtgggaaacgtttgagggcgaaactgtatacatgccggtacgcacatgggacgctaaaactggtaaagttggtaagttgtggggcgaaattaaataa

SEQ ID NO: 44 - protein, 280 aa, artificial
  artificial construct
MRGSHHHHHHGSGSGSGIEGRPYNGTGSACELAATHEHSAQWLNNYKKGYGYGPYPLGINGGMHYGVDFFMNIGTPVKAISSGKIVEAGWSNYGGGNQIGLIENDGVHRQWYMHLSKYNVKVGDYVKAGQIIGWSGSTGYSTAPHLHFQRMVNSFSNSTAQDPMPFLKSAGYGKAGGTVTPTPNTGWKQNKDGIWYKAEHASFTVTAPEGIITRYKGPWTGHPQAGVLQKGQTIKYDEVQKFDGHVWVSWETFEGETVYMPVRTWDAKTGKVGKLWGEIK

SEQ ID NO: 45 - DNA, 837 bp, artificial
  artificial construct
atgagaggatcgcatcaccatcaccatcacggatctggctctggatctggtatcgagggaaggccttataatggaactggatccgcatgcgagctcgctgcaacacatgaacattcagcacaatggttgaataattacaaaaaaggatatggttacggtccttatccattaggtataaatggcggtatgcactacggagttgatttttttatgaatattggaacaccagtaaaagctatttcaagcggaaaaatagttgaagctggttggagtaattacggaggaggtaatcaaataggtcttattgaaaatgatggagtgcatagacaatggtatatgcatctaagtaaatataatgttaaagtaggagattatgtcaaagctggtcaaataatcggttggtctggaagcactggttattctacagcaccacatttacacttccaaagaatggttaattcattttcaaattcaactgcccaagatccaatgcctttcttaaagagcgcaggatatggaaaagcaggtggtacagtaactccaacgccgaatacaggttggaaaacaaacaaatatggcacactatataaatcagagtcagctagcttcacacctaatacagatataataacaagaacgactggtccatttagaagcatgccgcagtcaggagtcttaaaagcaggtcaaacaattcattatgatgaagtgatgaaacaagacggtcatgtttgggtaggttatacaggtaacagtggccaacgtatttacttgcctgtaagaacatggaataaatctactaatactttaggtgttctttggggaactataaagtaa

SEQ ID NO: 46 - protein, 278 aa, artificial
  artificial construct
MRGSHHHHHHGSGSGSGIEGRPYNGTGSACELAATHEHSAQWLNNYKKGYGYGPYPLGINGGMHYGVDFFMNIGTPVKAISSGKIVEAGWSNYGGGNQIGLIENDGVHRQWYMHLSKYNVKVGDYVKAGQIIGWSGSTGYSTAPHLHFQRMVNSFSNSTAQDPMPFLKSAGYGKAGGTVTPTPNTGWKTNKYGTLYKSESASFTPNTDIITRTTGPFRSMPQSGVLKAGQTIHYDEVMKQDGHVWVGYTGNSGQRIYLPVRTWNKSTNTLGVLWGTIK

SEQ ID NO: 47 - DNA, 843 bp, artificial
  artificial construct
atgagaggatcgcatcaccatcaccatcacggatctggctctggatctggtatcgagggaaggccttataatggaactggatccgcatgcgagctcgctgcaacacatgaacattcagcacaatggttgaataattacaaaaaaggatatggttacggtccttatccattaggtataaatggcggtatgcactacggagttgatttttttatgaatattggaacaccagtaaaagctatttcaagcggaaaaatagttgaagctggttggagtaattacggaggaggtaatcaaataggtcttattgaaaatgatggagtgcatagacaatggtatatgcatctaagtaaatataatgttaaagtaggagattatgtcaaagctggtcaaataatcggttggtctggaagcactggttattctacagcaccacatttacacttccaaagaatggttaattcattttcaaattcaactgcccaagatccaatgcctttcttaaagagcgcaggatatggaaaagcaggtggtacagtaactccaacgccgaatacaggtggtaaatctgcaagtaaaataacagttggaagtaaagcgccttataaccttaaatggtcaaaaggtgcttattttaatgcgaaaatcgacggcttaggtgctacttcagccactagatacggtgataatcgtactaactatagattcgatgttggacaggctgtatacgcgcctggaacattaatatatgtgtttgaaattatagatggttggtgtcgcatttattggaacaatcataatgagtggatatggcatgagagattgattgtgaaagaagtgttttaa

SEQ ID NO: 48 - protein, 280 aa, artificial
  artificial construct
MRGSHHHHHHGSGSGSGIEGRPYNGTGSACELAATHEHSAQWLNNYKKGYGYGPYPLGINGGMHYGVDFFMNIGTPVKAISSGKIVEAGWSNYGGGNQIGLIENDGVHRQWYMHLSKYNVKVGDYVKAGQIIGWSGSTGYSTAPHLHFQRMVNSFSNSTAQDPMPFLKSAGYGKAGGTVTPTPNTGGKSASKITVGSKAPYNLKWSKGAYFNAKIDGLGATSATRYGDNRTNYRFDVGQAVYAPGTLIYVFEIIDGWCRIYWNNHNEWIWHERLIVKEVF

SEQ ID NO: 49 - DNA, 1755 bp, artificial
  artificial construct
atgagaggatcgcatcaccatcaccatcacggatctggctctggatctggtatcgagggaagggcaaagaaagatgaaaaatcacaagtatgtagtggtttggctatggaaaaatatgacattacaaatttaaatgctaaacaagataaatcaaagaatgggagcgtgaaagagttgaaacatatctattcaaaccatattaaaggtaacaagattacagcaccaaaacctagtattcaaggtgtggtcatccacaatgattatggtagtatgacacctagtcaatacttaccatggttatatgcacgtgagaataacggtacacacgttaacggttgggctagtgtttatgcaaatagaaacgaagtgctttggtatcatccgacagactacgtagagtggcattgtggtaatcaatgggcaaatgctaacttaatcggatttgaagtgtgtgagtcgtatcctggtagaatctcggacaaattattcttagaaaatgaagaagcgacattgaaagtagctgcggatgtgatgaagtcgtacggattaccagttaatcgcaacactgtacgtctgcataacgaattcttcggaacttcttgtccacatcgttcgtgggacttgcatgttggcaaaggtgagccttacacaactactaatattaataaaatgaaagactacttcatcaaacgcatcaaacattattatgacggtgagctcgcaaagaaagatgaaaaatcacaagtatgtagtggtttggctatggaaaaatatgacattacaaatttaaatgctaaacaagataaatcaaagaatgggagcgtgaaagagttgaaacatatctattcaaaccatattaaaggtaacaagattacagcaccaaaacctagtattcaaggtgtggtcatccacaatgattatggtagtatgacacctagtcaatacttaccatggttatatgcacgtgagaataacggtacacacgttaacggttgggctagtgtttatgcaaatagaaacgaagtgctttggtatcatccgacagactacgtagagtggcattgtggtaatcaatgggcaaatgctaacttaatcggatttgaagtgtgtgagtcgtatcctggtagaatctcggacaaattattcttagaaaatgaagaagcgacattgaaagtagctgcggatgtgatgaagtcgtacggattaccagttaatcgcaacactgtacgtctgcataacgaattcttcggaacttcttgtccacatcgttcgtgggacttgcatgttggcaaaggtgagccttacacaactactaatattaataaaatgaaagactacttcatcaaacgcatcaaacattattatgacggtggaaagctagaagtaagcaaagcagcaactatcaaacaatctgacgttaagcaagaagttaaaaagcaagaagcaaaacaaattgtgaaagcaacagattggaaacagaataaagatggcatttggtataaagctgaacatgcttcgttcacagtgacagcaccagagggaattatcacaagatacaaaggtccttggactggtcacccacaagctggtgtattacaaaaaggtcaaacgattaaatatgatgaggttcaaaaatttgacggtcatgtttgggtatcgtgggaaacgtttgagggcgaaactgtatacatgccggtacgcacatgggacgctaaaactggtaaagttggtaagttgtggggcgaaattaaataa

SEQ ID NO: 50 - protein, 584 aa, artificial
  artificial construct
MRGSHHHHHHGSGSGSGIEGRAKKDEKSQVCSGLAMEKYDITNLNAKQDKSKNGSVKELKHIYSNHIKGNKITAPKPSIQGVVIHNDYGSMTPSQYLPWLYARENNGTHVNGWASVYANRNEVLWYHPTDYVEWHCGNQWANANLIGFEVCESYPGRISDKLFLENEEATLKVAADVMKSYGLPVNRNTVRLHNEFFGTSCPHRSWDLHVGKGEPYTTTNINKMKDYFIKRIKHYYDGELAKKDEKSQVCSGLAMEKYDITNLNAKQDKSKNGSVKELKHIYSNHIKGNKITAPKPSIQGVVIHNDYGSMTPSQYLPWLYARENNGTHVNGWASVYANRNEVLWYHPTDYVEWHCGNQWANANLIGFEVCESYPGRISDKLFLENEEATLKVAADVMKSYGLPVNRNTVRLHNEFFGTSCPHRSWDLHVGKGEPYTTTNINKMKDYFIKRIKHYYDGGKLEVSKAATIKQSDVKQEVKKQEAKQIVKATDWKQNKDGIWYKAEHASFTVTAPEGIITRYKGPWTGHPQAGVLQKGQTIKYDEVQKFDGHVWVSWETFEGETVYMPVRTWDAKTGKVGKLWGEIK

SEQ ID NO: 51 - DNA, 1749 bp, artificial
  artificial construct
atgagaggatcgcatcaccatcaccatcacggatctggctctggatctggtatcgagggaagggcaaagaaagatgaaaaatcacaagtatgtagtggtttggctatggaaaaatatgacattacaaatttaaatgctaaacaagataaatcaaagaatgggagcgtgaaagagttgaaacatatctattcaaaccatattaaaggtaacaagattacagcaccaaaacctagtattcaaggtgtggtcatccacaatgattatggtagtatgacacctagtcaatacttaccatggttatatgcacgtgagaataacggtacacacgttaacggttgggctagtgtttatgcaaatagaaacgaagtgctttggtatcatccgacagactacgtagagtggcattgtggtaatcaatgggcaaatgctaacttaatcggatttgaagtgtgtgagtcgtatcctggtagaatctcggacaaattattcttagaaaatgaagaagcgacattgaaagtagctgcggatgtgatgaagtcgtacggattaccagttaatcgcaacactgtacgtctgcataacgaattcttcggaacttcttgtccacatcgttcgtgggacttgcatgttggcaaaggtgagccttacacaactactaatattaataaaatgaaagactacttcatcaaacgcatcaaacattattatgacggtgagctcgcaaagaaagatgaaaaatcacaagtatgtagtggtttggctatggaaaaatatgacattacaaatttaaatgctaaacaagataaatcaaagaatgggagcgtgaaagagttgaaacatatctattcaaaccatattaaaggtaacaagattacagcaccaaaacctagtattcaaggtgtggtcatccacaatgattatggtagtatgacacctagtcaatacttaccatggttatatgcacgtgagaataacggtacacacgttaacggttgggctagtgtttatgcaaatagaaacgaagtgctttggtatcatccgacagactacgtagagtggcattgtggtaatcaatgggcaaatgctaacttaatcggatttgaagtgtgtgagtcgtatcctggtagaatctcggacaaattattcttagaaaatgaagaagcgacattgaaagtagctgcggatgtgatgaagtcgtacggattaccagttaatcgcaacactgtacgtctgcataacgaattcttcggaacttcttgtccacatcgttcgtgggacttgcatgttggcaaaggtgagccttacacaactactaatattaataaaatgaaagactacttcatcaaacgcatcaaacattattatgacggtggaaagctagaagtaagcaaagcagcaactatcaaacaatctgacgttaagcaagaagttaaaaagcaagaagcaaaacaaattgtgaaagcaacagattggaaaacaaacaaatatggcacactatataaatcagagtcagctagcttcacacctaatacagatataataacaagaacgactggtccatttagaagcatgccgcagtcaggagtcttaaaagcaggtcaaacaattcattatgatgaagtgatgaaacaagacggtcatgtttgggtaggttatacaggtaacagtggccaacgtatttacttgcctgtaagaacatggaataaatctactaatactttaggtgttctttggggaactataaagtaa

SEQ ID NO: 52 - protein, 582 aa, artificial
  artificial construct
MRGSHHHHHHGSGSGSGIEGRAKKDEKSQVCSGLAMEKYDITNLNAKQDKSKNGSVKELKHIYSNHIKGNKITAPKPSIQGVVIHNDYGSMTPSQYLPWLYARENNGTHVNGWASVYANRNEVLWYHPTDYVEWHCGNQWANANLIGFEVCESYPGRISDKLFLENEEATLKVAADVMKSYGLPVNRNTVRLHNEFFGTSCPHRSWDLHVGKGEPYTTTNINKMKDYFIKRIKHYYDGELAKKDEKSQVCSGLAMEKYDITNLNAKQDKSKNGSVKELKHIYSNHIKGNKITAPKPSIQGVVIHNDYGSMTPSQYLPWLYARENNGTHVNGWASVYANRNEVLWYHPTDYVEWHCGNQWANANLIGFEVCESYPGRISDKLFLENEEATLKVAADVMKSYGLPVNRNTVRLHNEFFGTSCPHRSWDLHVGKGEPYTTTNINKMKDYFIKRIKHYYDGGKLEVSKAATIKQSDVKQEVKKQEAKQIVKATDWKTNKYGTLYKSESASFTPNTDIITRTTGPFRSMPQSGVLKAGQTIHYDEVMKQDGHVWVGYTGNSGQRIYLPVRTWNKSTNTLGVLWGTIK

SEQ ID NO: 53 - DNA, 1755 bp, artificial
  artificial construct
atgagaggatcgcatcaccatcaccatcacggatctggctctggatctggtatcgagggaagggcaaagaaagatgaaaaatcacaagtatgtagtggtttggctatggaaaaatatgacattacaaatttaaatgctaaacaagataaatcaaagaatgggagcgtgaaagagttgaaacatatctattcaaaccatattaaaggtaacaagattacagcaccaaaacctagtattcaaggtgtggtcatccacaatgattatggtagtatgacacctagtcaatacttaccatggttatatgcacgtgagaataacggtacacacgttaacggttgggctagtgtttatgcaaatagaaacgaagtgctttggtatcatccgacagactacgtagagtggcattgtggtaatcaatgggcaaatgctaacttaatcggatttgaagtgtgtgagtcgtatcctggtagaatctcggacaaattattcttagaaaatgaagaagcgacattgaaagtagctgcggatgtgatgaagtcgtacggattaccagttaatcgcaacactgtacgtctgcataacgaattcttcggaacttcttgtccacatcgttcgtgggacttgcatgttggcaaaggtgagccttacacaactactaatattaataaaatgaaagactacttcatcaaacgcatcaaacattattatgacggtgagctcgcaaagaaagatgaaaaatcacaagtatgtagtggtttggctatggaaaaatatgacattacaaatttaaatgctaaacaagataaatcaaagaatgggagcgtgaaagagttgaaacatatctattcaaaccatattaaaggtaacaagattacagcaccaaaacctagtattcaaggtgtggtcatccacaatgattatggtagtatgacacctagtcaatacttaccatggttatatgcacgtgagaataacggtacacacgttaacggttgggctagtgtttatgcaaatagaaacgaagtgctttggtatcatccgacagactacgtagagtggcattgtggtaatcaatgggcaaatgctaacttaatcggatttgaagtgtgtgagtcgtatcctggtagaatctcggacaaattattcttagaaaatgaagaagcgacattgaaagtagctgcggatgtgatgaagtcgtacggattaccagttaatcgcaacactgtacgtctgcataacgaattcttcggaacttcttgtccacatcgttcgtgggacttgcatgttggcaaaggtgagccttacacaactactaatattaataaaatgaaagactacttcatcaaacgcatcaaacattattatgacggtggaaagctagaagtaagcaaagcagcaactatcaaacaatctgacgttaagcaagaagttaaaaagcaagaagcaaaacaaattgtgaaagcaacagatggtaaatctgcaagtaaaataacagttggaagtaaagcgccttataaccttaaatggtcaaaaggtgcttattttaatgcgaaaatcgacggcttaggtgctacttcagccactagatacggtgataatcgtactaactatagattcgatgttggacaggctgtatacgcgcctggaacattaatatatgtgtttgaaattatagatggttggtgtcgcatttattggaacaatcataatgagtggatatggcatgagagattgattgtgaaagaagtgttttaa

SEQ ID NO: 54 - protein, 584 aa, artificial
  artificial construct
MRGSHHHHHHGSGSGSGIEGRAKKDEKSQVCSGLAMEKYDITNLNAKQDKSKNGSVKELKHIYSNHIKGNKITAPKPSIQGVVIHNDYGSMTPSQYLPWLYARENNGTHVNGWASVYANRNEVLWYHPTDYVEWHCGNQWANANLIGFEVCESYPGRISDKLFLENEEATLKVAADVMKSYGLPVNRNTVRLHNEFFGTSCPHRSWDLHVGKGEPYTTTNINKMKDYFIKRIKHYYDGELAKKDEKSQVCSGLAMEKYDITNLNAKQDKSKNGSVKELKHIYSNHIKGNKITAPKPSIQGVVIHNDYGSMTPSQYLPWLYARENNGTHVNGWASVYANRNEVLWYHPTDYVEWHCGNQWANANLIGFEVCESYPGRISDKLFLENEEATLKVAADVMKSYGLPVNRNTVRLHNEFFGTSCPHRSWDLHVGKGEPYTTTNINKMKDYFIKRIKHYYDGGKLEVSKAATIKQSDVKQEVKKQEAKQIVKATDGKSASKITVGSKAPYNLKWSKGAYFNAKIDGLGATSATRYGDNRTNYRFDVGQAVYAPGTLIYVFEIIDGWCRIYWNNHNEWIWHERLIVKEVF

SEQ ID NO: 55 - DNA, 1533 bp, artificial
  artificial construct
atgagaggatcgcatcaccatcaccatcacggatctggctctggatctggtatcgagggaaggatggctaagactcaagcagaaataaataaacgtttagatgcttatgcaaaaggaacagtagatagcccttacagagttaaaaaagctacaagttatgacccatcatttggtgtaatggaagcaggagccattgatgcagatggttactatcacgctcagtgtcaagaccttattacagactatgttttatggttaacagataataaagttagaacttggggtaatgctaaagaccaaattaaacagagttatggtactggatttaaaatacatgaaaataaaccttctactgtacctaaaaaaggttggattgcggtatttacatccggtagttatgaacagtggggtcacataggtattgtatatgatggaggtaatacttctacatttactattttagagcaaaactggaatggttatgctaataaaaaacctacaaaacgtgtagataattattacggattaactcacttcattgaaatacctgtaaaagcaggaactactgttaaaaaagaaacagctaagaaaagcgcaagtaaaacgcctgcacctaaaaagaaagcaacactaaaagtttctaagaatgagctcatggctaagactcaagcagaaataaataaacgtttagatgcttatgcaaaaggaacagtagatagcccttacagagttaaaaaagctacaagttatgacccatcatttggtgtaatggaagcaggagccattgatgcagatggttactatcacgctcagtgtcaagaccttattacagactatgttttatggttaacagataataaagttagaacttggggtaatgctaaagaccaaattaaacagagttatggtactggatttaaaatacatgaaaataaaccttctactgtacctaaaaaaggttggattgcggtatttacatccggtagttatgaacagtggggtcacataggtattgtatatgatggaggtaatacttctacatttactattttagagcaaaactggaatggttatgctaataaaaaacctacaaaacgtgtagataattattacggattaactcacttcattgaaatacctgtaaaagcaggaaagctagaagtaagcaaagcagcaactatcaaacaatctgacgttaagcaagaagttaaaaagcaagaagcaaaacaaattgtgaaagcaacagattggaaacagaataaagatggcatttggtataaagctgaacatgcttcgttcacagtgacagcaccagagggaattatcacaagatacaaaggtccttggactggtcacccacaagctggtgtattacaaaaaggtcaaacgattaaatatgatgaggttcaaaaatttgacggtcatgtttgggtatcgtgggaaacgtttgagggcgaaactgtatacatgccggtacgcacatgggacgctaaaactggtaaagttggtaagttgtggggcgaaattaaataa

SEQ ID NO: 56 - protein, 510 aa, artificial
  artificial construct
MRGSHHHHHHGSGSGSGIEGRMAKTQAEINKRLDAYAKGTVDSPYRVKKATSYDPSFGVMEAGAIDADGYYHAQCQDLITDYVLWLTDNKVRTWGNAKDQIKQSYGTGFKIHENKPSTVPKKGWIAVFTSGSYEQWGHIGIVYDGGNTSTFTILEQNWNGYANKKPTKRVDNYYGLTHFIEIPVKAGTTVKKETAKKSASKTPAPKKKATLKVSKNELMAKTQAEINKRLDAYAKGTVDSPYRVKKATSYDPSFGVMEAGAIDADGYYHAQCQDLITDYVLWLTDNKVRTWGNAKDQIKQSYGTGFKIHENKPSTVPKKGWIAVFTSGSYEQWGHIGIVYDGGNTSTFTILEQNWNGYANKKPTKRVDNYYGLTHFIEIPVKAGKLEVSKAATIKQSDVKQEVKKQEAKQIVKATDWKQNKDGIWYKAEHASFTVTAPEGIITRYKGPWTGHPQAGVLQKGQTIKYDEVQKFDGHVWVSWETFEGETVYMPVRTWDAKTGKVGKLWGEIK

SEQ ID NO: 57 - DNA, 1470 bp, artificial
  artificial construct
atgagaggatcgcatcaccatcaccatcacggatctggctctggatctggtatcgagggaaggatggctaagactcaagcagaaataaataaacgtttagatgcttatgcaaaaggaacagtagatagcccttacagagttaaaaaagctacaagttatgacccatcatttggtgtaatggaagcaggagccattgatgcagatggttactatcacgctcagtgtcaagaccttattacagactatgttttatggttaacagataataaagttagaacttggggtaatgctaaagaccaaattaaacagagttatggtactggatttaaaatacatgaaaataaaccttctactgtacctaaaaaaggttggattgcggtatttacatccggtagttatgaacagtggggtcacataggtattgtatatgatggaggtaatacttctacatttactattttagagcaaaactggaatggttatgctaataaaaaacctacaaaacgtgtagataattattacggattaactcacttcattgaaatacctgtaaaagcaggaactactgttaaaaaagaaacagctaagaaaagcgcaagtaaaacgcctgcacctaaaaagaaagcaacactaaaagtttctaagaatgagctcatggctaagactcaagcagaaataaataaacgtttagatgcttatgcaaaaggaacagtagatagcccttacagagttaaaaaagctacaagttatgacccatcatttggtgtaatggaagcaggagccattgatgcagatggttactatcacgctcagtgtcaagaccttattacagactatgttttatggttaacagataataaagttagaacttggggtaatgctaaagaccaaattaaacagagttatggtactggatttaaaatacatgaaaataaaccttctactgtacctaaaaaaggttggattgcggtatttacatccggtagttatgaacagtggggtcacataggtattgtatatgatggaggtaatacttctacatttactattttagagcaaaactggaatggttatgctaataaaaaacctacaaaacgtgtagataattattacggattaactcacttcattgaaatacctgtaaaagcaggaaaagcaggtggtacagtaactccaacgccgaatacaggttggaaaacaaacaaatatggcacactatataaatcagagtcagctagcttcacacctaatacagatataataacaagaacgactggtccatttagaagcatgccgcagtcaggagtcttaaaagcaggtcaaacaattcattatgatgaagtgatgaaacaagacggtcatgtttgggtaggttatacaggtaacagtggccaacgtatttacttgcctgtaagaacatggaataaatctactaatactttaggtgttctttggggaactataaagtaa

SEQ ID NO: 58 - protein, 489 aa, artificial
  artificial construct
MRGSHHHHHHGSGSGSGIEGRMAKTQAEINKRLDAYAKGTVDSPYRVKKATSYDPSFGVMEAGAIDADGYYHAQCQDLITDYVLWLTDNKVRTWGNAKDQIKQSYGTGFKIHENKPSTVPKKGWIAVFTSGSYEQWGHIGIVYDGGNTSTFTILEQNWNGYANKKPTKRVDNYYGLTHFIEIPVKAGTTVKKETAKKSASKTPAPKKKATLKVSKNELMAKTQAEINKRLDAYAKGTVDSPYRVKKATSYDPSFGVMEAGAIDADGYYHAQCQDLITDYVLWLTDNKVRTWGNAKDQIKQSYGTGFKIHENKPSTVPKKGWIAVFTSGSYEQWGHIGIVYDGGNTSTFTILEQNWNGYANKKPTKRVDNYYGLTHFIEIPVKAGKAGGTVTPTPNTGWKTNKYGTLYKSESASFTPNTDIITRTTGPFRSMPQSGVLKAGQTIHYDEVMKQDGHVWVGYTGNSGQRIYLPVRTWNKSTNTLGVLWGTIK

SEQ ID NO: 59 - DNA, 1524 bp, artificial
  artificial construct
atgagaggatcgcatcaccatcaccatcacggatctggctctggatctggtatcgagggaaggatggctaagactcaagcagaaataaataaacgtttagatgcttatgcaaaaggaacagtagatagcccttacagagttaaaaaagctacaagttatgacccatcatttggtgtaatggaagcaggagccattgatgcagatggttactatcacgctcagtgtcaagaccttattacagactatgttttatggttaacagataataaagttagaacttggggtaatgctaaagaccaaattaaacagagttatggtactggatttaaaatacatgaaaataaaccttctactgtacctaaaaaaggttggattgcggtatttacatccggtagttatgaacagtggggtcacataggtattgtatatgatggaggtaatacttctacatttactattttagagcaaaactggaatggttatgctaataaaaaacctacaaaacgtgtagataattattacggattaactcacttcattgaaatacctgtaaaagcaggaactactgttaaaaaagaaacagctaagaaaagcgcaagtaaaacgcctgcacctaaaaagaaagcaacactaaaagtttctaagaatgagctcatggctaagactcaagcagaaataaataaacgtttagatgcttatgcaaaaggaacagtagatagcccttacagagttaaaaaagctacaagttatgacccatcatttggtgtaatggaagcaggagccattgatgcagatggttactatcacgctcagtgtcaagaccttattacagactatgttttatggttaacagataataaagttagaacttggggtaatgctaaagaccaaattaaacagagttatggtactggatttaaaatacatgaaaataaaccttctactgtacctaaaaaaggttggattgcggtatttacatccggtagttatgaacagtggggtcacataggtattgtatatgatggaggtaatacttctacatttactattttagagcaaaactggaatggttatgctaataaaaaacctacaaaacgtgtagataattattacggattaactcacttcattgaaatacctgtaaaagcaggaactactgttaaaaaagaaacagctaagaaaagcgcaagtaaaacgcctgcacctaaaaagaaagcaacactaaaagtttctaagaatggtaaatctgcaagtaaaataacagttggaagtaaagcgccttataaccttaaatggtcaaaaggtgcttattttaatgcgaaaatcgacggcttaggtgctacttcagccactagatacggtgataatcgtactaactatagattcgatgttggacaggctgtatacgcgcctggaacattaatatatgtgtttgaaattatagatggttggtgtcgcatttattggaacaatcataatgagtggatatggcatgagagattgattgtgaaagaagtgttttaa

SEQ ID NO: 60 - protein, 507 aa, artificial
  artificial construct
MRGSHHHHHHGSGSGSGIEGRMAKTQAEINKRLDAYAKGTVDSPYRVKKATSYDPSFGVMEAGAIDADGYYHAQCQDLITDYVLWLTDNKVRTWGNAKDQIKQSYGTGFKIHENKPSTVPKKGWIAVFTSGSYEQWGHIGIVYDGGNTSTFTILEQNWNGYANKKPTKRVDNYYGLTHFIEIPVKAGTTVKKETAKKSASKTPAPKKKATLKVSKNELMAKTQAEINKRLDAYAKGTVDSPYRVKKATSYDPSFGVMEAGAIDADGYYHAQCQDLITDYVLWLTDNKVRTWGNAKDQIKQSYGTGFKIHENKPSTVPKKGWIAVFTSGSYEQWGHIGIVYDGGNTSTFTILEQNWNGYANKKPTKRVDNYYGLTHFIEIPVKAGTTVKKETAKKSASKTPAPKKKATLKVSKNGKSASKITVGSKAPYNLKWSKGAYFNAKIDGLGATSATRYGDNRTNYRFDVGQAVYAPGTLIYVFEIIDGWCRIYWNNHNEWIWHERLIVKEVF

SEQ ID NO: 61 - DNA, 1446 bp, artificial
  artificial construct
atgagaggatcgcatcaccatcaccatcacggatctggctctggatctggtatcgagggaaggatgaaaaccctgaaacaagcagagtcctacattaagagtaaagtaaatacaggaactgattttgatggtttatatgggtatcagtgtatggacttagcagtagattatatttaccatgtaacagatggtaaaataagaatgtggggtaatgctaaggatgcgataaataactcttttggtggtactgctacggtatataaaaactaccctgcttttagacctaagtacggtgatgtagtcgtatggactactggtaattttgcaacttatggtcatatcgcaatagttactaaccctgacccttatggagaccttcaatatgttacagttcttgaacaaaactggaacggtaacgggatttataaaaccgagttagctacaatcagaacacacgattacacaggaattacacattttattagacctaactttgctactgaatcaagtgtaaaaaagaaagatacaaagaaaaaaccaaaaccatcaaatagagatggaataaataaagataaaattgtatatgatagaactaatattaattacaatgagctcatgaaaaccctgaaacaagcagagtcctacattaagagtaaagtaaatacaggaactgattttgatggtttatatgggtatcagtgtatggacttagcagtagattatatttaccatgtaacagatggtaaaataagaatgtggggtaatgctaaggatgcgataaataactcttttggtggtactgctacggtatataaaaactaccctgcttttagacctaagtacggtgatgtagtcgtatggactactggtaattttgcaacttatggtcatatcgcaatagttactaaccctgacccttatggagaccttcaatatgttacagttcttgaacaaaactggaacggtaacgggatttataaaaccgagttagctacaatcagaacacacgattacacaggaattacacattttattagacctaactttgctactgaatcaagtgtaaaaaagaaagatacaaagaaaaaaccaaaaccatcaaatagagatggaataaataaagataaaattgtatatgatagaactaatattaattacaattggaaacagaataaagatggcatttggtataaagctgaacatgcttcgttcacagtgacagcaccagagggaattatcacaagatacaaaggtccttggactggtcacccacaagctggtgtattacaaaaaggtcaaacgattaaatatgatgaggttcaaaaatttgacggtcatgtttgggtatcgtgggaaacgtttgagggcgaaactgtatacatgccggtacgcacatgggacgctaaaactggtaaagttggtaagttgtggggcgaaattaaataa

SEQ ID NO: 62 - protein, 481 aa, artificial
  artificial construct
MRGSHHHHHHGSGSGSGIEGRMKTLKQAESYIKSKVNTGTDFDGLYGYQCMDLAVDYIYHVTDGKIRMWGNAKDAINNSFGGTATVYKNYPAFRPKYGDVVVWTTGNFATYGHIAIVTNPDPYGDLQYVTVLEQNWNGNGIYKTELATIRTHDYTGITHFIRPNFATESSVKKKDTKKKPKPSNRDGINKDKIVYDRTNINYNELMKTLKQAESYIKSKVNTGTDFDGLYGYQCMDLAVDYIYHVTDGKIRMWGNAKDAINNSFGGTATVYKNYPAFRPKYGDVVVWTTGNFATYGHIAIVTNPDPYGDLQYVTVLEQNWNGNGIYKTELATIRTHDYTGITHFIRPNFATESSVKKKDTKKKPKPSNRDGINKDKIVYDRTNINYNWKQNKDGIWYKAEHASFTVTAPEGIITRYKGPWTGHPQAGVLQKGQTIKYDEVQKFDGHVWVSWETFEGETVYMPVRTWDAKTGKVGKLWGEIK

SEQ ID NO: 63 - DNA, 1440 bp, artificial
  artificial construct
atgagaggatcgcatcaccatcaccatcacggatctggctctggatctggtatcgagggaaggatgaaaaccctgaaacaagcagagtcctacattaagagtaaagtaaatacaggaactgattttgatggtttatatgggtatcagtgtatggacttagcagtagattatatttaccatgtaacagatggtaaaataagaatgtggggtaatgctaaggatgcgataaataactcttttggtggtactgctacggtatataaaaactaccctgcttttagacctaagtacggtgatgtagtcgtatggactactggtaattttgcaacttatggtcatatcgcaatagttactaaccctgacccttatggagaccttcaatatgttacagttcttgaacaaaactggaacggtaacgggatttataaaaccgagttagctacaatcagaacacacgattacacaggaattacacattttattagacctaactttgctactgaatcaagtgtaaaaaagaaagatacaaagaaaaaaccaaaaccatcaaatagagatggaataaataaagataaaattgtatatgatagaactaatattaattacaatgagctcatgaaaaccctgaaacaagcagagtcctacattaagagtaaagtaaatacaggaactgattttgatggtttatatgggtatcagtgtatggacttagcagtagattatatttaccatgtaacagatggtaaaataagaatgtggggtaatgctaaggatgcgataaataactcttttggtggtactgctacggtatataaaaactaccctgcttttagacctaagtacggtgatgtagtcgtatggactactggtaattttgcaacttatggtcatatcgcaatagttactaaccctgacccttatggagaccttcaatatgttacagttcttgaacaaaactggaacggtaacgggatttataaaaccgagttagctacaatcagaacacacgattacacaggaattacacattttattagacctaactttgctactgaatcaagtgtaaaaaagaaagatacaaagaaaaaaccaaaaccatcaaatagagatggaataaataaagataaaattgtatatgatagaactaatattaattacaattggaaaacaaacaaatatggcacactatataaatcagagtcagctagcttcacacctaatacagatataataacaagaacgactggtccatttagaagcatgccgcagtcaggagtcttaaaagcaggtcaaacaattcattatgatgaagtgatgaaacaagacggtcatgtttgggtaggttatacaggtaacagtggccaacgtatttacttgcctgtaagaacatggaataaatctactaatactttaggtgttctttggggaactataaagtaa

SEQ ID NO: 64 - protein, 479 aa, artificial
  artificial construct
MRGSHHHHHHGSGSGSGIEGRMKTLKQAESYIKSKVNTGTDFDGLYGYQCMDLAVDYIYHVTDGKIRMWGNAKDAINNSFGGTATVYKNYPAFRPKYGDVVVWTTGNFATYGHIAIVTNPDPYGDLQYVTVLEQNWNGNGIYKTELATIRTHDYTGITHFIRPNFATESSVKKKDTKKKPKPSNRDGINKDKIVYDRTNINYNELMKTLKQAESYIKSKVNTGTDFDGLYGYQCMDLAVDYIYHVTDGKIRMWGNAKDAINNSFGGTATVYKNYPAFRPKYGDVVVWTTGNFATYGHIAIVTNPDPYGDLQYVTVLEQNWNGNGIYKTELATIRTHDYTGITHFIRPNFATESSVKKKDTKKKPKPSNRDGINKDKIVYDRTNINYNWKTNKYGTLYKSESASFTPNTDIITRTTGPFRSMPQSGVLKAGQTIHYDEVMKQDGHVWVGYTGNSGQRIYLPVRTWNKSTNTLGVLWGTIK

SEQ ID NO: 65 - DNA, 1446 bp, artificial
  artificial construct
atgagaggatcgcatcaccatcaccatcacggatctggctctggatctggtatcgagggaaggatgaaaaccctgaaacaagcagagtcctacattaagagtaaagtaaatacaggaactgattttgatggtttatatgggtatcagtgtatggacttagcagtagattatatttaccatgtaacagatggtaaaataagaatgtggggtaatgctaaggatgcgataaataactcttttggtggtactgctacggtatataaaaactaccctgcttttagacctaagtacggtgatgtagtcgtatggactactggtaattttgcaacttatggtcatatcgcaatagttactaaccctgacccttatggagaccttcaatatgttacagttcttgaacaaaactggaacggtaacgggatttataaaaccgagttagctacaatcagaacacacgattacacaggaattacacattttattagacctaactttgctactgaatcaagtgtaaaaaagaaagatacaaagaaaaaaccaaaaccatcaaatagagatggaataaataaagataaaattgtatatgatagaactaatattaattacaatgagctcatgaaaaccctgaaacaagcagagtcctacattaagagtaaagtaaatacaggaactgattttgatggtttatatgggtatcagtgtatggacttagcagtagattatatttaccatgtaacagatggtaaaataagaatgtggggtaatgctaaggatgcgataaataactcttttggtggtactgctacggtatataaaaactaccctgcttttagacctaagtacggtgatgtagtcgtatggactactggtaattttgcaacttatggtcatatcgcaatagttactaaccctgacccttatggagaccttcaatatgttacagttcttgaacaaaactggaacggtaacgggatttataaaaccgagttagctacaatcagaacacacgattacacaggaattacacattttattagacctaactttgctactgaatcaagtgtaaaaaagaaagatacaaagaaaaaaccaaaaccatcaaatagagatggaataaataaagataaaattgtatatgatagaactaatattaattacaatggtaaatctgcaagtaaaataacagttggaagtaaagcgccttataaccttaaatggtcaaaaggtgcttattttaatgcgaaaatcgacggcttaggtgctacttcagccactagatacggtgataatcgtactaactatagattcgatgttggacaggctgtatacgcgcctggaacattaatatatgtgtttgaaattatagatggttggtgtcgcatttattggaacaatcataatgagtggatatggcatgagagattgattgtgaaagaagtgttttaa

SEQ ID NO: 66 - protein, 481 aa, artificial
  artificial construct
MRGSHHHHHHGSGSGSGIEGRMKTLKQAESYIKSKVNTGTDFDGLYGYQCMDLAVDYIYHVTDGKIRMWGNAKDAINNSFGGTATVYKNYPAFRPKYGDVVVWTTGNFATYGHIAIVTNPDPYGDLQYVTVLEQNWNGNGIYKTELATIRTHDYTGITHFIRPNFATESSVKKKDTKKKPKPSNRDGINKDKIVYDRTNINYNELMKTLKQAESYIKSKVNTGTDFDGLYGYQCMDLAVDYIYHVTDGKIRMWGNAKDAINNSFGGTATVYKNYPAFRPKYGDVVVWTTGNFATYGHIAIVTNPDPYGDLQYVTVLEQNWNGNGIYKTELATIRTHDYTGITHFIRPNFATESSVKKKDTKKKPKPSNRDGINKDKIVYDRTNINYNGKSASKITVGSKAPYNLKWSKGAYFNAKIDGLGATSATRYGDNRTNYRFDVGQAVYAPGTLIYVFEIIDGWCRIYWNNHNEWIWHERLIVKEVF

SEQ ID NO: 67 - DNA, 1278 bp, artificial
  artificial construct
atgagaggatcgcatcaccatcaccatcacggatctggctctggatctggtatcgagggaagggctgcaacacatgaacattcagcacaatggttgaataattacaaaaaaggatatggttacggtccttatccattaggtataaatggcggtatgcactacggagttgatttttttatgaatattggaacaccagtaaaagctatttcaagcggaaaaatagttgaagctggttggagtaattacggaggaggtaatcaaataggtcttattgaaaatgatggagtgcatagacaatggtatatgcatctaagtaaatataatgttaaagtaggagattatgtcaaagctggtcaaataatcggttggtctggaagcactggttattctacagcaccacatttacacttccaaagaatggttaattcattttcaaattcaactgcccaagatccaatgcctttcttaaagagcgcaggatatggaaaagcaggtggtacagtaactccaacgccgaatacaggtgagctcgctgcaacacatgaacattcagcacaatggttgaataattacaaaaaaggatatggttacggtccttatccattaggtataaatggcggtatgcactacggagttgatttttttatgaatattggaacaccagtaaaagctatttcaagcggaaaaatagttgaagctggttggagtaattacggaggaggtaatcaaataggtcttattgaaaatgatggagtgcatagacaatggtatatgcatctaagtaaatataatgttaaagtaggagattatgtcaaagctggtcaaataatcggttggtctggaagcactggttattctacagcaccacatttacacttccaaagaatggttaattcattttcaaattcaactgcccaagatccaatgcctttcttaaagagcgcaggatatggaaaagcaggtggtacagtaactccaacgccgaatacaggttggaaacagaataaagatggcatttggtataaagctgaacatgcttcgttcacagtgacagcaccagagggaattatcacaagatacaaaggtccttggactggtcacccacaagctggtgtattacaaaaaggtcaaacgattaaatatgatgaggttcaaaaatttgacggtcatgtttgggtatcgtgggaaacgtttgagggcgaaactgtatacatgccggtacgcacatgggacgctaaaactggtaaagttggtaagttgtggggcgaaattaaataa

SEQ ID NO: 68 - protein, 425 aa, artificial
  artificial construct
MRGSHHHHHHGSGSGSGIEGRAATHEHSAQWLNNYKKGYGYGPYPLGINGGMHYGVDFFMNIGTPVKAISSGKIVEAGWSNYGGGNQIGLIENDGVHRQWYMHLSKYNVKVGDYVKAGQIIGWSGSTGYSTAPHLHFQRMVNSFSNSTAQDPMPFLKSAGYGKAGGTVTPTPNTGELAATHEHSAQWLNNYKKGYGYGPYPLGINGGMHYGVDFFMNIGTPVKAISSGKIVEAGWSNYGGGNQIGLIENDGVHRQWYMHLSKYNVKVGDYVKAGQIIGWSGSTGYSTAPHLHFQRMVNSFSNSTAQDPMPFLKSAGYGKAGGTVTPTPNTGWKQNKDGIWYKAEHASFTVTAPEGIITRYKGPWTGHPQAGVLQKGQTIKYDEVQKFDGHVWVSWETFEGETVYMPVRTWDAKTGKVGKLWGEIK

SEQ ID NO: 69 - DNA, 1272 bp, artificial
  artificial construct
atgagaggatcgcatcaccatcaccatcacggatctggctctggatctggtatcgagggaagggctgcaacacatgaacattcagcacaatggttgaataattacaaaaaaggatatggttacggtccttatccattaggtataaatggcggtatgcactacggagttgatttttttatgaatattggaacaccagtaaaagctatttcaagcggaaaaatagttgaagctggttggagtaattacggaggaggtaatcaaataggtcttattgaaaatgatggagtgcatagacaatggtatatgcatctaagtaaatataatgttaaagtaggagattatgtcaaagctggtcaaataatcggttggtctggaagcactggttattctacagcaccacatttacacttccaaagaatggttaattcattttcaaattcaactgcccaagatccaatgcctttcttaaagagcgcaggatatggaaaagcaggtggtacagtaactccaacgccgaatacaggtgagctcgctgcaacacatgaacattcagcacaatggttgaataattacaaaaaaggatatggttacggtccttatccattaggtataaatggcggtatgcactacggagttgatttttttatgaatattggaacaccagtaaaagctatttcaagcggaaaaatagttgaagctggttggagtaattacggaggaggtaatcaaataggtcttattgaaaatgatggagtgcatagacaatggtatatgcatctaagtaaatataatgttaaagtaggagattatgtcaaagctggtcaaataatcggttggtctggaagcactggttattctacagcaccacatttacacttccaaagaatggttaattcattttcaaattcaactgcccaagatccaatgcctttcttaaagagcgcaggatatggaaaagcaggtggtacagtaactccaacgccgaatacaggttggaaaacaaacaaatatggcacactatataaatcagagtcagctagcttcacacctaatacagatataataacaagaacgactggtccatttagaagcatgccgcagtcaggagtcttaaaagcaggtcaaacaattcattatgatgaagtgatgaaacaagacggtcatgtttgggtaggttatacaggtaacagtggccaacgtatttacttgcctgtaagaacatggaataaatctactaatactttaggtgttctttggggaactataaagtaa

SEQ ID NO: 70 - protein, 423 aa, artificial
  artificial construct
MRGSHHHHHHGSGSGSGIEGRAATHEHSAQWLNNYKKGYGYGPYPLGINGGMHYGVDFFMNIGTPVKAISSGKIVEAGWSNYGGGNQIGLIENDGVHRQWYMHLSKYNVKVGDYVKAGQIIGWSGSTGYSTAPHLHFQRMVNSFSNSTAQDPMPFLKSAGYGKAGGTVTPTPNTGELAATHEHSAQWLNNYKKGYGYGPYPLGINGGMHYGVDFFMNIGTPVKAISSGKIVEAGWSNYGGGNQIGLIENDGVHRQWYMHLSKYNVKVGDYVKAGQIIGWSGSTGYSTAPHLHFQRMVNSFSNSTAQDPMPFLKSAGYGKAGGTVTPTPNTGWKTNKYGTLYKSESASFTPNTDIITRTTGPFRSMPQSGVLKAGQTIHYDEVMKQDGHVWVGYTGNSGQRIYLPVRTWNKSTNTLGVLWGTIK

SEQ ID NO: 71 - DNA, 1278 bp, artificial
  artificial construct
atgagaggatcgcatcaccatcaccatcacggatctggctctggatctggtatcgagggaagggctgcaacacatgaacattcagcacaatggttgaataattacaaaaaaggatatggttacggtccttatccattaggtataaatggcggtatgcactacggagttgatttttttatgaatattggaacaccagtaaaagctatttcaagcggaaaaatagttgaagctggttggagtaattacggaggaggtaatcaaataggtcttattgaaaatgatggagtgcatagacaatggtatatgcatctaagtaaatataatgttaaagtaggagattatgtcaaagctggtcaaataatcggttggtctggaagcactggttattctacagcaccacatttacacttccaaagaatggttaattcattttcaaattcaactgcccaagatccaatgcctttcttaaagagcgcaggatatggaaaagcaggtggtacagtaactccaacgccgaatacaggtgagctcgctgcaacacatgaacattcagcacaatggttgaataattacaaaaaaggatatggttacggtccttatccattaggtataaatggcggtatgcactacggagttgatttttttatgaatattggaacaccagtaaaagctatttcaagcggaaaaatagttgaagctggttggagtaattacggaggaggtaatcaaataggtcttattgaaaatgatggagtgcatagacaatggtatatgcatctaagtaaatataatgttaaagtaggagattatgtcaaagctggtcaaataatcggttggtctggaagcactggttattctacagcaccacatttacacttccaaagaatggttaattcattttcaaattcaactgcccaagatccaatgcctttcttaaagagcgcaggatatggaaaagcaggtggtacagtaactccaacgccgaatacaggtggtaaatctgcaagtaaaataacagttggaagtaaagcgccttataaccttaaatggtcaaaaggtgcttattttaatgcgaaaatcgacggcttaggtgctacttcagccactagatacggtgataatcgtactaactatagattcgatgttggacaggctgtatacgcgcctggaacattaatatatgtgtttgaaattatagatggttggtgtcgcatttattggaacaatcataatgagtggatatggcatgagagattgattgtgaaagaagtgttttaa

SEQ ID NO: 72 - protein, 425 aa, artificial
  artificial construct
MRGSHHHHHHGSGSGSGIEGRAATHEHSAQWLNNYKKGYGYGPYPLGINGGMHYGVDFFMNIGTPVKAISSGKIVEAGWSNYGGGNQIGLIENDGVHRQWYMHLSKYNVKVGDYVKAGQIIGWSGSTGYSTAPHLHFQRMVNSFSNSTAQDPMPFLKSAGYGKAGGTVTPTPNTGELAATHEHSAQWLNNYKKGYGYGPYPLGINGGMHYGVDFFMNIGTPVKAISSGKIVEAGWSNYGGGNQIGLIENDGVHRQWYMHLSKYNVKVGDYVKAGQIIGWSGSTGYSTAPHLHFQRMVNSFSNSTAQDPMPFLKSAGYGKAGGTVTPTPNTGGKSASKITVGSKAPYNLKWSKGAYFNAKIDGLGATSATRYGDNRTNYRFDVGQAVYAPGTLIYVFEIIDGWCRIYWNNHNEWIWHERLIVKEVF

SEQ ID NO: 73 - DNA, 63 bp, artificial
  artificial his-tag
atgagaggatcgcatcaccatcaccatcacggatctggctctggatctggtatcgagggaagg

SEQ ID NO: 74 - protein, 21 aa, artificial
  artificial Hist-tag
MRGSHHHHHHGSGSGSGIEGR

SEQ ID NO: 75 - DNA, 741 bp, Staphylococcus simulans
gctgcaacacatgaacattcagcacaatggttgaataattacaaaaaaggatatggttacggtccttatccattaggtataaatggcggtatgcactacggagttgatttttttatgaatattggaacaccagtaaaagctatttcaagcggaaaaatagttgaagctggttggagtaattacggaggaggtaatcaaataggtcttattgaaaatgatggagtgcatagacaatggtatatgcatctaagtaaatataatgttaaagtaggagattatgtcaaagctggtcaaataatcggttggtctggaagcactggttattctacagcaccacatttacacttccaaagaatggttaattcattttcaaattcaactgcccaagatccaatgcctttcttaaagagcgcaggatatggaaaagcaggtggtacagtaactccaacgccgaatacaggttggaaaacaaacaaatatggcacactatataaatcagagtcagctagcttcacacctaatacagatataataacaagaacgactggtccatttagaagcatgccgcagtcaggagtcttaaaagcaggtcaaacaattcattatgatgaagtgatgaaacaagacggtcatgtttgggtaggttatacaggtaacagtggccaacgtatttacttgcctgtaagaacatggaataaatctactaatactttaggtgttctttggggaactataaagtga

SEQ ID NO: 76 - protein, 246 aa, Staphylococcus simulans
AATHEHSAQWLNNYKKGYGYGPYPLGINGGMHYGVDFFMNIGTPVKAISSGKIVEAGWSNYGGGNQIGLIENDGVHRQWYMHLSKYNVKVGDYVKAGQIIGWSGSTGYSTAPHLHFQRMVNSFSNSTAQDPMPFLKSAGYGKAGGTVTPTPNTGWKTNKYGTLYKSESASFTPNTDIITRTTGPFRSMPQSGVLKAGQTIHYDEVMKQDGHVWVGYTGNSGQRIYLPVRTWNKSTNTLGVLWGTIK

SEQ ID NO: 77 - DNA, 2019 bp, artificial
  artificial construct
atgagaggatcgcatcaccatcaccatcacggatccatgcaagcaaaattaactaaaaatgagtttatagagtggttgaaaacttctgagggaaaacaattcaatgtggacttatggtatggatttcaatgctttgattatgccaatgctggttggaaagttttgtttggattacttctaaaaggtttaggtgcaaaagatattccgttcgctaacaacttcgacggattagctactgtataccaaaatacaccggacttcttagcacaacctggcgacatggtggtattcggtagcaactacggtgctggatatggtcacgttgcatgggtaattgaagcaactttagattacatcattgtatatgagcagaattggctaggcggtggctggactgacggaatcgaacaacccggctggggttgggaaaaagttacaagacgacaacatgcttatgatttccctatgtggtttatccgtccgaattttaaaagtgagacagcgccacgatcagttcaatctcctacacaagcacctaaaaaagaaacagctggatccatgctaactgctattgactatcttacgaaaaaaggttggaaaatatcatctgaccctcgcacttacgatggttaccctaaaaactacggctacagaaattaccatgaaaacggcattaattatgatgagttttgtggtggttatcatagagcttttgatgtttacagtaacgaaactaacgacgtgcctgctgttactagcggaacagttattgaagcaaacgattacggtaattttggtggtacattcgttattagagacgctaacgataacgattggatatatgggcatctacaacgtggctcaatgcgatttgttgtaggcgacaaagtcaatcaaggtgacattattggtttacaaggtaatagcaactattacgacaatcctatgagtgtacatttacatttacaattacgccctaaagacgcaaagaaagatgaaaaatcacaagtatgtagtggtttggctatggaaaaatatgacattacaaatttaaatgctaaacaagataaatcaaagaatgggagcgtgaaagagttgaaacatatctattcaaaccatattaaaggtaacaagattacagcaccaaaacctagtattcaaggtgtggtcatccacaatgattatggtagtatgacacctagtcaatacttaccatggttatatgcacgtgagaataacggtacacacgttaacggttgggctagtgtttatgcaaatagaaacgaagtgctttggtatcatccgacagactacgtagagtggcattgtggtaatcaatgggcaaatgctaacttaatcggatttgaagtgtgtgagtcgtatcctggtagaatctcggacaaattattcttagaaaatgaagaagcgacattgaaagtagctgcggatgtgatgaagtcgtacggattaccagttaatcgcaacactgtacgtctgcataacgaattcttcggaacttcttgtccacatcgttcgtgggacttgcatgttggcaaaggtgagccttacacaactactaatattaataaaatgaaagactacttcatcaaacgcatcaaacattattatgacggtggaaagctagaagtaagcaaagcagcaactatcaaacaatctgacgttaagcaagaagttaaaaagcaagaagcaaaacaaattgtgaaagcaacagattggaaacagaataaagatggcatttggtataaagctgaacatgcttcgttcacagtgacagcaccagagggaattatcacaagatacaaaggtccttggactggtcacccacaagctggtgtattacaaaaaggtcaaacgattaaatatgatgaggttcaaaaatttgacggtcatgtttgggtatcgtgggaaacgtttgagggcgaaactgtatacatgccggtacgcacatgggacgctaaaactggtaaagttggtaagttgtggggcgaaattaaataa

SEQ ID NO: 78 - protein, 672 aa, artificial
  artificial construct
MRGSHHHHHHGSMQAKLTKNEFIEWLKTSEGKQFNVDLWYGFQCFDYANAGWKVLFGLLLKGLGAKDIPFANNFDGLATVYQNTPDFLAQPGDMVVFGSNYGAGYGHVAWVIEATLDYIIVYEQNWLGGGWTDGIEQPGWGWEKVTRRQHAYDFPMWFIRPNFKSETAPRSVQSPTQAPKKETAGSMLTAIDYLTKKGWKISSDPRTYDGYPKNYGYRNYHENGINYDEFCGGYHRAFDVYSNETNDVPAVTSGTVIEANDYGNFGGTFVIRDANDNDWIYGHLQRGSMRFVVGDKVNQGDIIGLQGNSNYYDNPMSVHLHLQLRPKDAKKDEKSQVCSGLAMEKYDITNLNAKQDKSKNGSVKELKHIYSNHIKGNKITAPKPSIQGVVIHNDYGSMTPSQYLPWLYARENNGTHVNGWASVYANRNEVLWYHPTDYVEWHCGNQWANANLIGFEVCESYPGRISDKLFLENEEATLKVAADVMKSYGLPVNRNTVRLHNEFFGTSCPHRSWDLHVGKGEPYTTTNINKMKDYFIKRIKHYYDGGKLEVSKAATIKQSDVKQEVKKQEAKQIVKATDWKQNKDGIWYKAEHASFTVTAPEGIITRYKGPWTGHPQAGVLQKGQTIKYDEVQKFDGHVWVSWETFEGETVYMPVRTWDAKTGKVGKLWGEIK

SEQ ID NO: 79 - DNA, 2145 bp, artificial
  artificial construct
atgagaggatcgcatcaccatcaccatcacggatccaagccacaacctaaagcagtagaacttaaaatcatcaaagatgtggttaaaggttatgacctacctaagcgtggtagtaaccctaaaggtatagttatacacaacgacgcagggagcaaaggggcgactgctgaagcatatcgtaacggattagtaaatgcacctttatcaagattagaagcgggcattgcgcatagttacgtatcaggcaacacagtttggcaagccttagatgaatcacaagtaggttggcataccgctaatcaaataggtaataaatattattacggtattgaagtatgtcaatcaatgggcgcagataacgcgacattcttaaaaaatgaacaggcaactttccaagaatgcgctagattgttgaaaaaatggggattaccagcaaacagaaatacaatcagattgcacaatgaatttacttcaacatcatgccctcatagaagttcggttttacacactggttttgacccagtaactcgcggtctattgccagaagacaagcggttgcaacttaaagactactttatcaagcagattagggcgtacatggatggtaaaataccggttgccactgtctctaatgagtcaagcgcttcaagtaatacagttaaaccagttgcaagtgcaggatccatgctaactgctattgactatcttacgaaaaaaggttggaaaatatcatctgaccctcgcacttacgatggttaccctaaaaactacggctacagaaattaccatgaaaacggcattaattatgatgagttttgtggtggttatcatagagcttttgatgtttacagtaacgaaactaacgacgtgcctgctgttactagcggaacagttattgaagcaaacgattacggtaattttggtggtacattcgttattagagacgctaacgataacgattggatatatgggcatctacaacgtggctcaatgcgatttgttgtaggcgacaaagtcaatcaaggtgacattattggtttacaaggtaatagcaactattacgacaatcctatgagtgtacatttacatttacaattacgccctaaagacgcaaagaaagatgaaaaatcacaagtatgtagtggtttggctatggaaaaatatgacattacaaatttaaatgctaaacaagataaatcaaagaatgggagcgtgaaagagttgaaacatatctattcaaaccatattaaaggtaacaagattacagcaccaaaacctagtattcaaggtgtggtcatccacaatgattatggtagtatgacacctagtcaatacttaccatggttatatgcacgtgagaataacggtacacacgttaacggttgggctagtgtttatgcaaatagaaacgaagtgctttggtatcatccgacagactacgtagagtggcattgtggtaatcaatgggcaaatgctaacttaatcggatttgaagtgtgtgagtcgtatcctggtagaatctcggacaaattattcttagaaaatgaagaagcgacattgaaagtagctgcggatgtgatgaagtcgtacggattaccagttaatcgcaacactgtacgtctgcataacgaattcttcggaacttcttgtccacatcgttcgtgggacttgcatgttggcaaaggtgagccttacacaactactaatattaataaaatgaaagactacttcatcaaacgcatcaaacattattatgacggtggaaagctagaagtaagcaaagcagcaactatcaaacaatctgacgttaagcaagaagttaaaaagcaagaagcaaaacaaattgtgaaagcaacagattggaaacagaataaagatggcatttggtataaagctgaacatgcttcgttcacagtgacagcaccagagggaattatcacaagatacaaaggtccttggactggtcacccacaagctggtgtattacaaaaaggtcaaacgattaaatatgatgaggttcaaaaatttgacggtcatgtttgggtatcgtgggaaacgtttgagggcgaaactgtatacatgccggtacgcacatgggacgctaaaactggtaaagttggtaagttgtggggcgaaattaaataa

SEQ ID NO: 80 - protein, 714 aa, artificial
  artificial construct
MRGSHHHHHHGSKPQPKAVELKIIKDVVKGYDLPKRGSNPKGIVIHNDAGSKGATAEAYRNGLVNAPLSRLEAGIAHSYVSGNTVWQALDESQVGWHTANQIGNKYYYGIEVCQSMGADNATFLKNEQATFQECARLLKKWGLPANRNTIRLHNEFTSTSCPHRSSVLHTGFDPVTRGLLPEDKRLQLKDYFIKQIRAYMDGKIPVATVSNESSASSNTVKPVASAGSMLTAIDYLTKKGWKISSDPRTYDGYPKNYGYRNYHENGINYDEFCGGYHRAFDVYSNETNDVPAVTSGTVIEANDYGNFGGTFVIRDANDNDWIYGHLQRGSMRFVVGDKVNQGDIIGLQGNSNYYDNPMSVHLHLQLRPKDAKKDEKSQVCSGLAMEKYDITNLNAKQDKSKNGSVKELKHIYSNHIKGNKITAPKPSIQGVVIHNDYGSMTPSQYLPWLYARENNGTHVNGWASVYANRNEVLWYHPTDYVEWHCGNQWANANLIGFEVCESYPGRISDKLFLENEEATLKVAADVMKSYGLPVNRNTVRLHNEFFGTSCPHRSWDLHVGKGEPYTTTNINKMKDYFIKRIKHYYDGGKLEVSKAATIKQSDVKQEVKKQEAKQIVKATDWKQNKDGIWYKAEHASFTVTAPEGIITRYKGPWTGHPQAGVLQKGQTIKYDEVQKFDGHVWVSWETFEGETVYMPVRTWDAKTGKVGKLWGEIK

SEQ ID NO: 81 - DNA, 1959 bp, artificial
  artificial construct
atgagaggatcgcatcaccatcaccatcacggatccatgaaaaccctgaaacaagcagagtcctacattaagagtaaagtaaatacaggaactgattttgatggtttatatgggtatcagtgtatggacttagcagtagattatatttaccatgtaacagatggtaaaataagaatgtggggtaatgctaaggatgcgataaataactcttttggtggtactgctacggtatataaaaactaccctgcttttagacctaagtacggtgatgtagtcgtatggactactggtaattttgcaacttatggtcatatcgcaatagttactaaccctgacccttatggagaccttcaatatgttacagttcttgaacaaaactggaacggtaacgggatttataaaaccgagttagctacaatcagaacacacgattacacaggaattacacattttattaaagacgcaaagaaagatgaaaaatcacaagtatgtagtggtttggctatggaaaaatatgacattacaaatttaaatgctaaacaagataaatcaaagaatgggagcgtgaaagagttgaaacatatctattcaaaccatattaaaggtaacaagattacagcaccaaaacctagtattcaaggtgtggtcatccacaatgattatggtagtatgacacctagtcaatacttaccatggttatatgcacgtgagaataacggtacacacgttaacggttgggctagtgtttatgcaaatagaaacgaagtgctttggtatcatccgacagactacgtagagtggcattgtggtaatcaatgggcaaatgctaacttaatcggatttgaagtgtgtgagtcgtatcctggtagaatctcggacaaattattcttagaaaatgaagaagcgacattgaaagtagctgcggatgtgatgaagtcgtacggattaccagttaatcgcaacactgtacgtctgcataacgaattcttcggaacttcttgtccacatcgttcgtgggacttgcatgttggcaaaggtgagccttacacaactactaatattaataaaatgaaagactacttcatcaaacgcatcaaacattattatgacggtggaaagctagaagtaagcaaagcagcaactatcaaacaatctgacgttaagcaagaagttaaaaagcaagaagcaaaacaaattgtgaaagcaacagatgctgcaacacatgaacattcagcacaatggttgaataattacaaaaaaggatatggttacggtccttatccattaggtataaatggcggtatgcactacggagttgatttttttatgaatattggaacaccagtaaaagctatttcaagcggaaaaatagttgaagctggttggagtaattacggaggaggtaatcaaataggtcttattgaaaatgatggagtgcatagacaatggtatatgcatctaagtaaatataatgttaaagtaggagattatgtcaaagctggtcaaataatcggttggtctggaagcactggttattctacagcaccacatttacacttccaaagaatggttaattcattttcaaattcaactgcccaagatccaatgcctttcttaaagagcgcaggatatggaaaagcaggtggtacagtaactccaacgccgaatacaggttggaaacagaataaagatggcatttggtataaagctgaacatgcttcgttcacagtgacagcaccagagggaattatcacaagatacaaaggtccttggactggtcacccacaagctggtgtattacaaaaaggtcaaacgattaaatatgatgaggttcaaaaatttgacggtcatgtttgggtatcgtgggaaacgtttgagggcgaaactgtatacatgccggtacgcacatgggacgctaaaactggtaaagttggtaagttgtggggcgaaattaaataa

SEQ ID NO: 82 - protein, 652 aa, artificial
  artificial construct
MRGSHHHHHHGSMKTLKQAESYIKSKVNTGTDFDGLYGYQCMDLAVDYIYHVTDGKIRMWGNAKDAINNSFGGTATVYKNYPAFRPKYGDVVVWTTGNFATYGHIAIVTNPDPYGDLQYVTVLEQNWNGNGIYKTELATIRTHDYTGITHFIKDAKKDEKSQVCSGLAMEKYDITNLNAKQDKSKNGSVKELKHIYSNHIKGNKITAPKPSIQGVVIHNDYGSMTPSQYLPWLYARENNGTHVNGWASVYANRNEVLWYHPTDYVEWHCGNQWANANLIGFEVCESYPGRISDKLFLENEEATLKVAADVMKSYGLPVNRNTVRLHNEFFGTSCPHRSWDLHVGKGEPYTTTNINKMKDYFIKRIKHYYDGGKLEVSKAATIKQSDVKQEVKKQEAKQIVKATDAATHEHSAQWLNNYKKGYGYGPYPLGINGGMHYGVDFFMNIGTPVKAISSGKIVEAGWSNYGGGNQIGLIENDGVHRQWYMHLSKYNVKVGDYVKAGQIIGWSGSTGYSTAPHLHFQRMVNSFSNSTAQDPMPFLKSAGYGKAGGTVTPTPNTGWKQNKDGIWYKAEHASFTVTAPEGIITRYKGPWTGHPQAGVLQKGQTIKYDEVQKFDGHVWVSWETFEGETVYMPVRTWDAKTGKVGKLWGEIK

SEQ ID NO: 83 - DNA, 1554 bp, artificial
  artificial construct
atgagaggatcgcatcaccatcaccatcacggatccgctgcaacacatgaacattcagcacaatggttgaataattacaaaaaaggatatggttacggtccttatccattaggtataaatggcggtatgcactacggagttgatttttttatgaatattggaacaccagtaaaagctatttcaagcggaaaaatagttgaagctggttggagtaattacggaggaggtaatcaaataggtcttattgaaaatgatggagtgcatagacaatggtatatgcatctaagtaaatataatgttaaagtaggagattatgtcaaagctggtcaaataatcggttggtctggaagcactggttattctacagcaccacatttacacttccaaagaatggttaattcattttcaaattcaactgcccaagatccaatgcctttcttaaagagcgcaggatatggaaaagcaggtggtacagtaactccaacgccgaatacaggtgagctcttacgccctaaagacgcaaagaaagatgaaaaatcacaagtatgtagtggtttggctatggaaaaatatgacattacaaatttaaatgctaaacaagataaatcaaagaatgggagcgtgaaagagttgaaacatatctattcaaaccatattaaaggtaacaagattacagcaccaaaacctagtattcaaggtgtggtcatccacaatgattatggtagtatgacacctagtcaatacttaccatggttatatgcacgtgagaataacggtacacacgttaacggttgggctagtgtttatgcaaatagaaacgaagtgctttggtatcatccgacagactacgtagagtggcattgtggtaatcaatgggcaaatgctaacttaatcggatttgaagtgtgtgagtcgtatcctggtagaatctcggacaaattattcttagaaaatgaagaagcgacattgaaagtagctgcggatgtgatgaagtcgtacggattaccagttaatcgcaacactgtacgtctgcataacgaattcttcggaacttcttgtccacatcgttcgtgggacttgcatgttggcaaaggtgagccttacacaactactaatattaataaaatgaaagactacttcatcaaacgcatcaaacattattatgacggtggaaagctagaagtaagcaaagcagcaactatcaaacaatctgacgttaagcaagaagttaaaaagcaagaagcaaaacaaattgtgaaagcaacagattggaaacagaataaagatggcatttggtataaagctgaacatgcttcgttcacagtgacagcaccagagggaattatcacaagatacaaaggtccttggactggtcacccacaagctggtgtattacaaaaaggtcaaacgattaaatatgatgaggttcaaaaatttgacggtcatgtttgggtatcgtgggaaacgtttgagggcgaaactgtatacatgccggtacgcacatgggacgctaaaactggtaaagttggtaagttgtggggcgaaattaaataa

SEQ ID NO: 84 - protein, 517 aa, artificial
  artificial construct
MRGSHHHHHHGSAATHEHSAQWLNNYKKGYGYGPYPLGINGGMHYGVDFFMNIGTPVKAISSGKIVEAGWSNYGGGNQIGLIENDGVHRQWYMHLSKYNVKVGDYVKAGQIIGWSGSTGYSTAPHLHFQRMVNSFSNSTAQDPMPFLKSAGYGKAGGTVTPTPNTGELLRPKDAKKDEKSQVCSGLAMEKYDITNLNAKQDKSKNGSVKELKHIYSNHIKGNKITAPKPSIQGVVIHNDYGSMTPSQYLPWLYARENNGTHVNGWASVYANRNEVLWYHPTDYVEWHCGNQWANANLIGFEVCESYPGRISDKLFLENEEATLKVAADVMKSYGLPVNRNTVRLHNEFFGTSCPHRSWDLHVGKGEPYTTTNINKMKDYFIKRIKHYYDGGKLEVSKAATIKQSDVKQEVKKQEAKQIVKATDWKQNKDGIWYKAEHASFTVTAPEGIITRYKGPWTGHPQAGVLQKGQTIKYDEVQKFDGHVWVSWETFEGETVYMPVRTWDAKTGKVGKLWGEIK

SEQ ID NO: 85 - DNA, 1887 bp, artificial
  artificial construct
atgagaggatcgcatcaccatcaccatcacggatccatgctaactgctattgactatcttacgaaaaaaggttggaaaatatcatctgaccctcgcacttacgatggttaccctaaaaactacggctacagaaattaccatgaaaacggcattaattatgatgagttttgtggtggttatcatagagcttttgatgtttacagtaacgaaactaacgacgtgcctgctgttactagcggaacagttattgaagcaaacgattacggtaattttggtggtacattcgttattagagacgctaacgataacgattggatatatgggcatctacaacgtggctcaatgcgatttgttgtaggcgacaaagtcaatcaaggtgacattattggtttacaaggtaatagcaactattacgacaatcctatgagtgtacatttacatttacaattacgccctaaagacgcaaagaaagatgaaaaatcacaagtatgtagtggtttggctatggaaaaatatgacattacaaatttaaatgctaaacaagataaatcaaagaatgggagcgtgaaagagttgaaacatatctattcaaaccatattaaaggtaacaagattacagcaccaaaacctagtattcaaggtgtggtcatccacaatgattatggtagtatgacacctagtcaatacttaccatggttatatgcacgtgagaataacggtacacacgttaacggttgggctagtgtttatgcaaatagaaacgaagtgctttggtatcatccgacagactacgtagagtggcattgtggtaatcaatgggcaaatgctaacttaatcggatttgaagtgtgtgagtcgtatcctggtagaatctcggacaaattattcttagaaaatgaagaagcgacattgaaagtagctgcggatgtgatgaagtcgtacggattaccagttaatcgcaacactgtacgtctgcataacgaattcttcggaacttcttgtccacatcgttcgtgggacttgcatgttggcaaaggtgagccttacacaactactaatattaataaaatgaaagactacttcatcaaacgcatcaaacattattatgacggtggaaagctagaagtaagcaaagcagcaactatcaaacaatctgacgttaagcaagaagttaaaaagcaagaagcaaaacaaattgtgaaagcaacagattggaaacagaataaagatggcatttggtataaagctgaacatgcttcgttcacagtgacagcaccagagggaattatcacaagatacaaaggtccttggactggtcacccacaagctggtgtattacaaaaaggtcaaacgattaaatatgatgaggttcaaaaatttgacggtcatgtttgggtatcgtgggaaacgtttgagggcgaaactgtatacatgccggtacgcacatgggacgctaaaactggtaaagttggtaagttgtggggcgaaattaaagagctcggtggaaagctagaagtaagcaaagcagcaactatcaaacaatctgacgttaagcaagaagttaaaaagcaagaagcaaaacaaattgtgaaagcaacagattggaaacagaataaagatggcatttggtataaagctgaacatgcttcgttcacagtgacagcaccagagggaattatcacaagatacaaaggtccttggactggtcacccacaagctggtgtattacaaaaaggtcaaacgattaaatatgatgaggttcaaaaatttgacggtcatgtttgggtatcgtgggaaacgtttgagggcgaaactgtatacatgccggtacgcacatgggacgctaaaactggtaaagttggtaagttgtggggcgaaattaaataa

SEQ ID NO: 86 - protein, 628 aa, artificial
  artificial construct
MRGSHHHHHHGSMLTAIDYLTKKGWKISSDPRTYDGYPKNYGYRNYHENGINYDEFCGGYHRAFDVYSNETNDVPAVTSGTVIEANDYGNFGGTFVIRDANDNDWIYGHLQRGSMRFVVGDKVNQGDIIGLQGNSNYYDNPMSVHLHLQLRPKDAKKDEKSQVCSGLAMEKYDITNLNAKQDKSKNGSVKELKHIYSNHIKGNKITAPKPSIQGVVIHNDYGSMTPSQYLPWLYARENNGTHVNGWASVYANRNEVLWYHPTDYVEWHCGNQWANANLIGFEVCESYPGRISDKLFLENEEATLKVAADVMKSYGLPVNRNTVRLHNEFFGTSCPHRSWDLHVGKGEPYTTTNINKMKDYFIKRIKHYYDGGKLEVSKAATIKQSDVKQEVKKQEAKQIVKATDWKQNKDGIWYKAEHASFTVTAPEGIITRYKGPWTGHPQAGVLQKGQTIKYDEVQKFDGHVWVSWETFEGETVYMPVRTWDAKTGKVGKLWGEIKELGGKLEVSKAATIKQSDVKQEVKKQEAKQIVKATDWKQNKDGIWYKAEHASFTVTAPEGIITRYKGPWTGHPQAGVLQKGQTIKYDEVQKFDGHVWVSWETFEGETVYMPVRTWDAKTGKVGKLWGEIK

SEQ ID NO: 87 - DNA, 1035 bp, artificial
  artificial construct
atgagaggatcgcatcaccatcaccatcacggatccatgctaactgctattgactatcttacgaaaaaaggttggaaaatatcatctgaccctcgcacttacgatggttaccctaaaaactacggctacagaaattaccatgaaaacggcattaattatgatgagttttgtggtggttatcatagagcttttgatgtttacagtaacgaaactaacgacgtgcctgctgttactagcggaacagttattgaagcaaacgattacggtaattttggtggtacattcgttattagagacgctaacgataacgattggatatatgggcatctacaacgtggctcaatgcgatttgttgtaggcgacaaagtcaatcaaggtgacattattggtttacaaggtaatagcaactattacgacaatcctatgagtgtacatttacatttacaattacgccctaaagacgcaaagaaagatgaaaaatcacaagtatgtagtggtttggctatggaaaaatatgacattacaaatttaaatgctaaacaagataaatcaaagaatgggagcgtgaaagagttgaaacatatctattcaaaccatattaaaggtaacaagattacagcaccaaaacctagtattcaaggtgagctcggtggaaagctagaagtaagcaaagcagcaactatcaaacaatctgacgttaagcaagaagttaaaaagcaagaagcaaaacaaattgtgaaagcaacagattggaaacagaataaagatggcatttggtataaagctgaacatgcttcgttcacagtgacagcaccagagggaattatcacaagatacaaaggtccttggactggtcacccacaagctggtgtattacaaaaaggtcaaacgattaaatatgatgaggttcaaaaatttgacggtcatgtttgggtatcgtgggaaacgtttgagggcgaaactgtatacatgccggtacgcacatgggacgctaaaactggtaaagttggtaagttgtggggcgaaattaaataa

SEQ ID NO: 88 - protein, 344 aa, artificial
  artificial construct
MRGSHHHHHHGSMLTAIDYLTKKGWKISSDPRTYDGYPKNYGYRNYHENGINYDEFCGGYHRAFDVYSNETNDVPAVTSGTVIEANDYGNFGGTFVIRDANDNDWIYGHLQRGSMRFVVGDKVNQGDIIGLQGNSNYYDNPMSVHLHLQLRPKDAKKDEKSQVCSGLAMEKYDITNLNAKQDKSKNGSVKELKHIYSNHIKGNKITAPKPSIQGELGGKLEVSKAATIKQSDVKQEVKKQEAKQIVKATDWKQNKDGIWYKAEHASFTVTAPEGIITRYKGPWTGHPQAGVLQKGQTIKYDEVQKFDGHVWVSWETFEGETVYMPVRTWDAKTGKVGKLWGEIK

SEQ ID NO: 89 - DNA, 2961 bp, artificial
  artificial construct
atgagaggatcgcatcaccatcaccatcacggatccatgctaactgctattgactatcttacgaaaaaaggttggaaaatatcatctgaccctcgcacttacgatggttaccctaaaaactacggctacagaaattaccatgaaaacggcattaattatgatgagttttgtggtggttatcatagagcttttgatgtttacagtaacgaaactaacgacgtgcctgctgttactagcggaacagttattgaagcaaacgattacggtaattttggtggtacattcgttattagagacgctaacgataacgattggatatatgggcatctacaacgtggctcaatgcgatttgttgtaggcgacaaagtcaatcaaggtgacattattggtttacaaggtaatagcaactattacgacaatcctatgagtgtacatttacatttacaattacgccctaaagacgcaaagaaagatgaaaaatcacaagtatgtagtggtttggctatggaaaaatatgacattacaaatttaaatgctaaacaagataaatcaaagaatgggagcgtgaaagagttgaaacatatctattcaaaccatattaaaggtaacaagattacagcaccaaaacctagtattcaaggtgtggtcatccacaatgattatggtagtatgacacctagtcaatacttaccatggttatatgcacgtgagaataacggtacacacgttaacggttgggctagtgtttatgcaaatagaaacgaagtgctttggtatcatccgacagactacgtagagtggcattgtggtaatcaatgggcaaatgctaacttaatcggatttgaagtgtgtgagtcgtatcctggtagaatctcggacaaattattcttagaaaatgaagaagcgacattgaaagtagctgcggatgtgatgaagtcgtacggattaccagttaatcgcaacactgtacgtctgcataacgaattcttcggaacttcttgtccacatcgttcgtgggacttgcatgttggcaaaggtgagccttacacaactactaatattaataaaatgaaagactacttcatcaaacgcatcaaacattattatgacggtggaaagctagaagtaagcaaagcagcaactatcaaacaatctgacgttaagcaagaagttaaaaagcaagaagcaaaacaaattgtgaaagcaacagattggaaacagaataaagatggcatttggtataaagctgaacatgcttcgttcacagtgacagcaccagagggaattatcacaagatacaaaggtccttggactggtcacccacaagctggtgtattacaaaaaggtcaaacgattaaatatgatgaggttcaaaaatttgacggtcatgtttgggtatcgtgggaaacgtttgagggcgaaactgtatacatgccggtacgcacatgggacgctaaaactggtaaagttggtaagttgtggggcgaaattaaagagctcatgctaactgctattgactatcttacgaaaaaaggttggaaaatatcatctgaccctcgcacttacgatggttaccctaaaaactacggctacagaaattaccatgaaaacggcattaattatgatgagttttgtggtggttatcatagagcttttgatgtttacagtaacgaaactaacgacgtgcctgctgttactagcggaacagttattgaagcaaacgattacggtaattttggtggtacattcgttattagagacgctaacgataacgattggatatatgggcatctacaacgtggctcaatgcgatttgttgtaggcgacaaagtcaatcaaggtgacattattggtttacaaggtaatagcaactattacgacaatcctatgagtgtacatttacatttacaattacgccctaaagacgcaaagaaagatgaaaaatcacaagtatgtagtggtttggctatggaaaaatatgacattacaaatttaaatgctaaacaagataaatcaaagaatgggagcgtgaaagagttgaaacatatctattcaaaccatattaaaggtaacaagattacagcaccaaaacctagtattcaaggtgtggtcatccacaatgattatggtagtatgacacctagtcaatacttaccatggttatatgcacgtgagaataacggtacacacgttaacggttgggctagtgtttatgcaaatagaaacgaagtgctttggtatcatccgacagactacgtagagtggcattgtggtaatcaatgggcaaatgctaacttaatcggatttgaagtgtgtgagtcgtatcctggtagaatctcggacaaattattcttagaaaatgaagaagcgacattgaaagtagctgcggatgtgatgaagtcgtacggattaccagttaatcgcaacactgtacgtctgcataacgaattcttcggaacttcttgtccacatcgttcgtgggacttgcatgttggcaaaggtgagccttacacaactactaatattaataaaatgaaagactacttcatcaaacgcatcaaacattattatgacggtggaaagctagaagtaagcaaagcagcaactatcaaacaatctgacgttaagcaagaagttaaaaagcaagaagcaaaacaaattgtgaaagcaacagattggaaacagaataaagatggcatttggtataaagctgaacatgcttcgttcacagtgacagcaccagagggaattatcacaagatacaaaggtccttggactggtcacccacaagctggtgtattacaaaaaggtcaaacgattaaatatgatgaggttcaaaaatttgacggtcatgtttgggtatcgtgggaaacgtttgagggcgaaactgtatacatgccggtacgcacatgggacgctaaaactggtaaagttggtaagttgtggggcgaaattaaataa

SEQ ID NO: 90 - protein, 986 aa, artificial
  artificial construct
MRGSHHHHHHGSMLTAIDYLTKKGWKISSDPRTYDGYPKNYGYRNYHENGINYDEFCGGYHRAFDVYSNETNDVPAVTSGTVIEANDYGNFGGTFVIRDANDNDWIYGHLQRGSMRFVVGDKVNQGDIIGLQGNSNYYDNPMSVHLHLQLRPKDAKKDEKSQVCSGLAMEKYDITNLNAKQDKSKNGSVKELKHIYSNHIKGNKITAPKPSIQGVVIHNDYGSMTPSQYLPWLYARENNGTHVNGWASVYANRNEVLWYHPTDYVEWHCGNQWANANLIGFEVCESYPGRISDKLFLENEEATLKVAADVMKSYGLPVNRNTVRLHNEFFGTSCPHRSWDLHVGKGEPYTTTNINKMKDYFIKRIKHYYDGGKLEVSKAATIKQSDVKQEVKKQEAKQIVKATDWKQNKDGIWYKAEHASFTVTAPEGIITRYKGPWTGHPQAGVLQKGQTIKYDEVQKFDGHVWVSWETFEGETVYMPVRTWDAKTGKVGKLWGEIKELMLTAIDYLTKKGWKISSDPRTYDGYPKNYGYRNYHENGINYDEFCGGYHRAFDVYSNETNDVPAVTSGTVIEANDYGNFGGTFVIRDANDNDWIYGHLQRGSMRFVVGDKVNQGDIIGLQGNSNYYDNPMSVHLHLQLRPKDAKKDEKSQVCSGLAMEKYDITNLNAKQDKSKNGSVKELKHIYSNHIKGNKITAPKPSIQGVVIHNDYGSMTPSQYLPWLYARENNGTHVNGWASVYANRNEVLWYHPTDYVEWHCGNQWANANLIGFEVCESYPGRISDKLFLENEEATLKVAADVMKSYGLPVNRNTVRLHNEFFGTSCPHRSWDLHVGKGEPYTTTNINKMKDYFIKRIKHYYDGGKLEVSKAATIKQSDVKQEVKKQEAKQIVKATDWKQNKDGIWYKAEHASFTVTAPEGIITRYKGPWTGHPQAGVLQKGQTIKYDEVQKFDGHVWVSWETFEGETVYMPVRTWDAKTGKVGKLWGEIK

SEQ ID NO: 91 - DNA, 1953 bp, artificial
  artificial construct
atgagaggatcgcatcaccatcaccatcacggatccatgaaaaccctgaaacaagcagagtcctacattaagagtaaagtaaatacaggaactgattttgatggtttatatgggtatcagtgtatggacttagcagtagattatatttaccatgtaacagatggtaaaataagaatgtggggtaatgctaaggatgcgataaataactcttttggtggtactgctacggtatataaaaactaccctgcttttagacctaagtacggtgatgtagtcgtatggactactggtaattttgcaacttatggtcatatcgcaatagttactaaccctgacccttatggagaccttcaatatgttacagttcttgaacaaaactggaacggtaacgggatttataaaaccgagttagctacaatcagaacacacgattacacaggaattacacattttattaaagacgcaaagaaagatgaaaaatcacaagtatgtagtggtttggctatggaaaaatatgacattacaaatttaaatgctaaacaagataaatcaaagaatgggagcgtgaaagagttgaaacatatctattcaaaccatattaaaggtaacaagattacagcaccaaaacctagtattcaaggtgtggtcatccacaatgattatggtagtatgacacctagtcaatacttaccatggttatatgcacgtgagaataacggtacacacgttaacggttgggctagtgtttatgcaaatagaaacgaagtgctttggtatcatccgacagactacgtagagtggcattgtggtaatcaatgggcaaatgctaacttaatcggatttgaagtgtgtgagtcgtatcctggtagaatctcggacaaattattcttagaaaatgaagaagcgacattgaaagtagctgcggatgtgatgaagtcgtacggattaccagttaatcgcaacactgtacgtctgcataacgaattcttcggaacttcttgtccacatcgttcgtgggacttgcatgttggcaaaggtgagccttacacaactactaatattaataaaatgaaagactacttcatcaaacgcatcaaacattattatgacggtggaaagctagaagtaagcaaagcagcaactatcaaacaatctgacgttaagcaagaagttaaaaagcaagaagcaaaacaaattgtgaaagcaacagatgctgcaacacatgaacattcagcacaatggttgaataattacaaaaaaggatatggttacggtccttatccattaggtataaatggcggtatgcactacggagttgatttttttatgaatattggaacaccagtaaaagctatttcaagcggaaaaatagttgaagctggttggagtaattacggaggaggtaatcaaataggtcttattgaaaatgatggagtgcatagacaatggtatatgcatctaagtaaatataatgttaaagtaggagattatgtcaaagctggtcaaataatcggttggtctggaagcactggttattctacagcaccacatttacacttccaaagaatggttaattcattttcaaattcaactgcccaagatccaatgcctttcttaaagagcgcaggatatggaaaagcaggtggtacagtaactccaacgccgaatacaggttggaaaacaaacaaatatggcacactatataaatcagagtcagctagcttcacacctaatacagatataataacaagaacgactggtccatttagaagcatgccgcagtcaggagtcttaaaagcaggtcaaacaattcattatgatgaagtgatgaaacaagacggtcatgtttgggtaggttatacaggtaacagtggccaacgtatttacttgcctgtaagaacatggaataaatctactaatactttaggtgttctttggggaactataaagtaa

SEQ ID NO: 92 - protein, 650 aa, artificial
  artificial construct
MRGSHHHHHHGSMKTLKQAESYIKSKVNTGTDFDGLYGYQCMDLAVDYIYHVTDGKIRMWGNAKDAINNSFGGTATVYKNYPAFRPKYGDVVVWTTGNFATYGHIAIVTNPDPYGDLQYVTVLEQNWNGNGIYKTELATIRTHDYTGITHFIKDAKKDEKSQVCSGLAMEKYDITNLNAKQDKSKNGSVKELKHIYSNHIKGNKITAPKPSIQGVVIHNDYGSMTPSQYLPWLYARENNGTHVNGWASVYANRNEVLWYHPTDYVEWHCGNQWANANLIGFEVCESYPGRISDKLFLENEEATLKVAADVMKSYGLPVNRNTVRLHNEFFGTSCPHRSWDLHVGKGEPYTTTNINKMKDYFIKRIKHYYDGGKLEVSKAATIKQSDVKQEVKKQEAKQIVKATDAATHEHSAQWLNNYKKGYGYGPYPLGINGGMHYGVDFFMNIGTPVKAISSGKIVEAGWSNYGGGNQIGLIENDGVHRQWYMHLSKYNVKVGDYVKAGQIIGWSGSTGYSTAPHLHFQRMVNSFSNSTAQDPMPFLKSAGYGKAGGTVTPTPNTGWKTNKYGTLYKSESASFTPNTDIITRTTGPFRSMPQSGVLKAGQTIHYDEVMKQDGHVWVGYTGNSGQRIYLPVRTWNKSTNTLGVLWGTIK

SEQ ID NO: 93 - DNA, 1521 bp, artificial
  artificial construct
atgagaggatcgcatcaccatcaccatcacggatccgctgcaacacatgaacattcagcacaatggttgaataattacaaaaaaggatatggttacggtccttatccattaggtataaatggcggtatgcactacggagttgatttttttatgaatattggaacaccagtaaaagctatttcaagcggaaaaatagttgaagctggttggagtaattacggaggaggtaatcaaataggtcttattgaaaatgatggagtgcatagacaatggtatatgcatctaagtaaatataatgttaaagtaggagattatgtcaaagctggtcaaataatcggttggtctggaagcactggttattctacagcaccacatttacacttccaaagaatggttaattcattttcaaattcaactgcccaagatccaatgcctttcttaaagagcgcaggatatggaaaagcaggtggtacagtaactccaacgccgaatacaggttggaaaacaaacaaatatggcacactatataaatcagagtcagctagcttcacacctaatacagatataataacaagaacgactggtccatttagaagcatgccgcagtcaggagtcttaaaagcaggtcaaacaattcattatgatgaagtgatgaaacaagacggtcatgtttgggtaggttatacaggtaacagtggccaacgtatttacttgcctgtaagaacatggaataaatctactaatactttaggtgttctttggggaactataaaggagctcgctgcaacacatgaacattcagcacaatggttgaataattacaaaaaaggatatggttacggtccttatccattaggtataaatggcggtatgcactacggagttgatttttttatgaatattggaacaccagtaaaagctatttcaagcggaaaaatagttgaagctggttggagtaattacggaggaggtaatcaaataggtcttattgaaaatgatggagtgcatagacaatggtatatgcatctaagtaaatataatgttaaagtaggagattatgtcaaagctggtcaaataatcggttggtctggaagcactggttattctacagcaccacatttacacttccaaagaatggttaattcattttcaaattcaactgcccaagatccaatgcctttcttaaagagcgcaggatatggaaaagcaggtggtacagtaactccaacgccgaatacaggttggaaaacaaacaaatatggcacactatataaatcagagtcagctagcttcacacctaatacagatataataacaagaacgactggtccatttagaagcatgccgcagtcaggagtcttaaaagcaggtcaaacaattcattatgatgaagtgatgaaacaagacggtcatgtttgggtaggttatacaggtaacagtggccaacgtatttacttgcctgtaagaacatggaataaatctactaatactttaggtgttctttggggaactataaagtga

SEQ ID NO: 94 - protein, 506 aa, artificial
  artificial construct
MRGSHHHHHHGSAATHEHSAQWLNNYKKGYGYGPYPLGINGGMHYGVDFFMNIGTPVKAISSGKIVEAGWSNYGGGNQIGLIENDGVHRQWYMHLSKYNVKVGDYVKAGQIIGWSGSTGYSTAPHLHFQRMVNSFSNSTAQDPMPFLKSAGYGKAGGTVTPTPNTGWKTNKYGTLYKSESASFTPNTDIITRTTGPFRSMPQSGVLKAGQTIHYDEVMKQDGHVWVGYTGNSGQRIYLPVRTWNKSTNTLGVLWGTIKELAATHEHSAQWLNNYKKGYGYGPYPLGINGGMHYGVDFFMNIGTPVKAISSGKIVEAGWSNYGGGNQIGLIENDGVHRQWYMHLSKYNVKVGDYVKAGQIIGWSGSTGYSTAPHLHFQRMVNSFSNSTAQDPMPFLKSAGYGKAGGTVTPTPNTGWKTNKYGTLYKSESASFTPNTDIITRTTGPFRSMPQSGVLKAGQTIHYDEVMKQDGHVWVGYTGNSGQRIYLPVRTWNKSTNTLGVLWGTIK

SEQ ID NO: 95 - DNA, 1143 bp, artificial
  artificial construct
atgagaggatcgcatcaccatcaccatcacggatccatgagtaaaggagaagaacttttcactggagttgtcccaattcttgttgaattagatggtgatgttaatgggcacaaattttctgtcagtggagagggtgaaggtgatgcaacatacggaaaacttacccttaaatttatttgcactactggaaaactacctgttccatggccaacacttgtcactactttcgcgtatggtcttcaatgctttgcgagatacccagatcatatgaaacggcatgactttttcaagagtgccatgcccgaaggttatgtacaggaaagaactatatttttcaaagatgacgggaactacaagacacgtgctgaagtcaagtttgaaggtgatacccttgttaatagaatcgagttaaaaggtattgattttaaagaagatggaaacattcttggacacaaattggaatacaactataactcacacaatgtatacatcatggcagacaaacaaaagaatggaatcaaagttaacttcaaaattagacacaacattgaagatggaagcgttcaactagcagaccattatcaacaaaatactccaattggcgatggccctgtccttttaccagacaaccattacctgtccacacaatctgccctttcgaaagatcccaacgaaaagagagaccacatggtccttcttgagtttgtaacagctgctgggattacacatggcatggatgaactatacaaagagctcggtggaaagctagaagtaagcaaagcagcaactatcaaacaatctgacgttaagcaagaagttaaaaagcaagaagcaaaacaaattgtgaaagcaacagattggaaacagaataaagatggcatttggtataaagctgaacatgcttcgttcacagtgacagcaccagagggaattatcacaagatacaaaggtccttggactggtcacccacaagctggtgtattacaaaaaggtcaaacgattaaatatgatgaggttcaaaaatttgacggtcatgtttgggtatcgtgggaaacgtttgagggcgaaactgtatacatgccggtacgcacatgggacgctaaaactggtaaagttggtaagttgtggggcgaaattaaataa

SEQ ID NO: 96 - protein, 380 aa, artificial
  artificial construct
MRGSHHHHHHGSMSKGEELFTGVVPILVELDGDVNGHKFSVSGEGEGDATYGKLTLKFICTTGKLPVPWPTLVTTFAYGLQCFARYPDHMKRHDFFKSAMPEGYVQERTIFFKDDGNYKTRAEVKFEGDTLVNRIELKGIDFKEDGNILGHKLEYNYNSHNVYIMADKQKNGIKVNFKIRHNIEDGSVQLADHYQQNTPIGDGPVLLPDNHYLSTQSALSKDPNEKRDHMVLLEFVTAAGITHGMDELYKELGGKLEVSKAATIKQSDVKQEVKKQEAKQIVKATDWKQNKDGIWYKAEHASFTVTAPEGIITRYKGPWTGHPQAGVLQKGQTIKYDEVQKFDGHVWVSWETFEGETVYMPVRTWDAKTGKVGKLWGEIK

SEQ ID NO: 97 - DNA, 516 bp, Staphylococcus bacteriophage phi 11
atgcaagcaaaattaactaaaaatgagtttatagagtggttgaaaacttctgagggaaaacaattcaatgtggacttatggtatggatttcaatgctttgattatgccaatgctggttggaaagttttgtttggattacttctaaaaggtttaggtgcaaaagatattccgttcgctaacaacttcgacggattagctactgtataccaaaatacaccggacttcttagcacaacctggcgacatggtggtattcggtagcaactacggtgctggatatggtcacgttgcatgggtaattgaagcaactttagattacatcattgtatatgagcagaattggctaggcggtggctggactgacggaatcgaacaacccggctggggttgggaaaaagttacaagacgacaacatgcttatgatttccctatgtggtttatccgtccgaattttaaaagtgagacagcgccacgatcagttcaatctcctacacaagcacctaaaaaagaaacagct

SEQ ID NO: 98 - protein, 158 aa, Staphylococcus bacteriophage phi 11
MSIIMEVATMQAKLTKNEFIEWLKTSEGKQFNVDLWYGFQCFDYANAGWKVLFGLLLKGLGAKDIPFANNFDGLATVYQNTPDFLAQPGDMVVFGSNYGAGYGHVAWVIEATLDYIIVYEQNWLGGGWTDGIEQPGWGWEKVTRRQHAYDFPMWFIRP

SEQ ID NO: 99 - DNA, 642 bp, Staphylococcus bacteriophage phi 11
aagccacaacctaaagcagtagaacttaaaatcatcaaagatgtggttaaaggttatgacctacctaagcgtggtagtaaccctaaaggtatagttatacacaacgacgcagggagcaaaggggcgactgctgaagcatatcgtaacggattagtaaatgcacctttatcaagattagaagcgggcattgcgcatagttacgtatcaggcaacacagtttggcaagccttagatgaatcacaagtaggttggcataccgctaatcaaataggtaataaatattattacggtattgaagtatgtcaatcaatgggcgcagataacgcgacattcttaaaaaatgaacaggcaactttccaagaatgcgctagattgttgaaaaaatggggattaccagcaaacagaaatacaatcagattgcacaatgaatttacttcaacatcatgccctcatagaagttcggttttacacactggttttgacccagtaactcgcggtctattgccagaagacaagcggttgcaacttaaagactactttatcaagcagattagggcgtacatggatggtaaaataccggttgccactgtctctaatgagtcaagcgcttcaagtaatacagttaaaccagttgcaagtgca

SEQ ID NO: 100 - protein, 163 aa, Staphylococcus bacteriophage phi 11
NPKGIVIHNDAGSKGATAEAYRNGLVNAPLSRLEAGIAHSYVSGNTVWQALDESQVGWHTANQIGNKYYYGIEVCQSMGADNATFLKNEQATFQECARLLKKWGLPANRNTIRLHNEFTSTSCPHRSSVLHTGFDPVTRGLLPEDKRLQLKDYFIKQIRAYMD

SEQ ID NO: 101 - protein, 462 aa, Artificial Sequence
  Synthetic construct
MAATHEHSAQWLNNYKKGYGYGPYPLGINGGMHYGVDFFMNIGTPVKAISSGKIVEAGWSNYGGGNQIGLIENDGVHRQWYMHLSKYNVKVGDYVKAGQIIGWSGSTGYSTAPHLHFQRMVNSFSNSTAQDPMPFLKSAGYGKAGGTVTPTPNTGLKHIYSNHIKGNKITAPKPSIQGVVIHNDYGSMTPSQYLPWLYARENNGTHVNGWASVYANRNEVLWYHPTDYVEWHCGNQWANANLIGFEVCESYPGRISDKLFLENEEATLKVAADVMKSYGLPVNRNTVRLHNEFFGTSCPHRSWDLHVGKGEPYTTTNINKMKDYFIKRIKHYYDGGKLEVSKAATIKQSDVKQEVKKQEAKQIVKATDWKQNKDGIWYKAEHASFTVTAPEGIITRYKGPWTGHPQAGVLQKGQTIKYDEVQKFDGHVWVSWETFEGETVYMPVRTWDAKTGKVGKLWGEIK